European Patent Application EP 4 316 507 A1, published February 7, 2024. Title: Composition for the preventing or treating cancer comprising an expression vector for dual genes. Applicant: YD LIFE SCIENCE CO., LTD Korea Research Institute of Bioscience and Biotechnology. The sequence listing filed with the application follows.

SEQUENCE LISTING (45 sequences)

SEQ ID NO: 1 - protein, 301 aa, Artificial Sequence
  CYB5R3 amino acid
MGAQLSTLGHMVLFPVWFLYSLLMKLFQRSTPAITLESPDIKYPLRLIDREIISHDTRRFRFALPSPQHILGLPVGQHIYLSARIDGNLVVRPYTPISSDDDKGFVDLVIKVYFKDTHPKFPAGGKMSQYLESMQIGDTIEFRGPSGLLVYQGKGKFAIRPDKKSNPIIRTVKSVGMIAGGTGITPMLQVIRAIMKDPDDHTVCHLLFANQTEKDILLRPELEELRNKHSARFKLWYTLDRAPEAWDYGQGFVNEEMIRDHLPPPEEEPLVLMCGPPPMIQYACLPNLDHVGHPTERCFVF

SEQ ID NO: 2 - DNA, 903 bp, Artificial Sequence
  CYB5R3 nucleotide
atgggggcccagctcagcacgttgggccatatggtgctcttcccagtctggttcctgtacagtctgctcatgaagctgttccagcgctccacgccagccatcaccctcgagagcccggacatcaagtatcctctcagactcatcgacagagagatcattagccatgacaccagaaggttcagatttgccctgccttcaccccagcacatcctgggcctccctgtcggccagcacatctacctctcggctcgaattgatggaaacctggtcgtccggccctatacacccatctccagcgatgatgacaagggcttcgtggacctggtcatcaaggtttacttcaaggacacccatcccaagtttcccgctggagggaagatgtctcagtacctggagagcatgcagattggagacaccattgagttccggggccccagtgggctgctggtctaccagggcaaagggaagttcgccatccgacctgacaaaaagtccaaccctatcatcaggacagtgaagtctgtgggcatgatcgcgggagggacaggcatcaccccgatgctgcaggtgatccgcgccatcatgaaggaccctgatgaccacactgtgtgccacctgctctttgccaaccagaccgagaaggacatcctgctgcgacctgagctggaggaactcaggaacaaacattctgcacgcttcaagctctggtacacgctggacagagcccctgaagcctgggactacggccagggcttcgtgaatgaggagatgatccgggaccaccttccacctccagaggaggagcctctggtgctgatgtgtggacctccacctatgatccagtacgcctgccttcccaacctggaccacgtgggccaccccacggagcgctgcttcgtcttc

SEQ ID NO: 3 - protein, 10 aa, Artificial Sequence
  HA amino acid
AYPYDVPDYA

SEQ ID NO: 4 - DNA, 30 bp, Artificial Sequence
  HA nucleotide
gcctacccttacgacgtcccagactacgct

SEQ ID NO: 5 - protein, 22 aa, Artificial Sequence
  CS amino acid
GSGATNFSLLKQAGDVEENPGP

SEQ ID NO: 6 - DNA, 66 bp, Artificial Sequence
  CS nucleotide
ggaagcggagctactaacttcagcctgctgaagcaggctggagacgtggaggagaaccctggacct

SEQ ID NO: 7 - protein, 10 aa, Artificial Sequence
  FLAG amino acid
GDYKDDDDKA

SEQ ID NO: 8 - DNA, 30 bp, Artificial Sequence
  FLAG nucleotide
ggagactacaaggacgacgatgacaaggct

SEQ ID NO: 9 - protein, 153 aa, Artificial Sequence
  IL-2 amino acid
MYRMQLLSCIALSLALVTNSAPTSSSTKKTQLQLEHLLLDLQMILNGINNYKNPKLTRMLTFKFYMPKKATELKHLQCLEEELKPLEEVLNLAQSKNFHLRPRDLISNINVIVLELKGSETTFMCEYADETATIVEFLNRWITFCQSIISTLT

SEQ ID NO: 10 - DNA, 459 bp, Artificial Sequence
  IL-2 nucleotide
atgtacaggatgcaactcctgtcttgcattgcactaagtcttgcacttgtcacaaacagtgcacctacttcaagttctacaaagaaaacacagctacaactggagcatttactgctggatttacagatgattttgaatggaattaataattacaagaatcccaaactcaccaggatgctcacatttaagttttacatgcccaagaaggccacagaactgaaacatcttcagtgtctagaagaagaactcaaacctctggaggaagtgctaaatttagctcaaagcaaaaactttcacttaagacccagggacttaatcagcaatatcaacgtaatagttctggaactaaagggatctgaaacaacattcatgtgtgaatatgctgatgagacagcaaccattgtagaatttctgaacagatggattaccttttgtcaaagcatcatctcaacactgact

SEQ ID NO: 11 - protein, 177 aa, Artificial Sequence
  IL-7 amino acid
MFHVSFRYIFGLPPLILVLLPVASSDCDIEGKDGKQYESVLMVSIDQLLDSMKEIGSNCLNNEFNFFKRHICDANKEGMFLFRAARKLRQFLKMNSTGDFDLHLLKVSEGTTILLNCTGQVKGRKPAALGEAQPTKSLEENKSLKEQKKLNDLCFLKRLLQEIKTCWNKILMGTKEH

SEQ ID NO: 12 - DNA, 531 bp, Artificial Sequence
  IL-7 nucleotide
atgttccatgtttcttttaggtatatctttggacttcctcccctgatccttgttctgttgccagtagcatcatctgattgtgatattgaaggtaaagatggcaaacaatatgagagtgttctaatggtcagcatcgatcaattattggacagcatgaaagaaattggtagcaattgcctgaataatgaatttaacttttttaaaagacatatctgtgatgctaataaggaaggtatgtttttattccgtgctgctcgcaagttgaggcaatttcttaaaatgaatagcactggtgattttgatctccacttattaaaagtttcagaaggcacaacaatactgttgaactgcactggccaggttaaaggaagaaaaccagctgccctgggtgaagcccaaccaacaaagagtttggaagaaaataaatctttaaaggaacagaaaaaactgaatgacttgtgtttcctaaagagactattacaagagataaaaacttgttggaataaaattttgatgggcactaaagaacac

SEQ ID NO: 13 - protein, 328 aa, Artificial Sequence
  IL-12B amino acid
MCHQQLVISWFSLVFLASPLVAIWELKKDVYVVELDWYPDAPGEMVVLTCDTPEEDGITWTLDQSSEVLGSGKTLTIQVKEFGDAGQYTCHKGGEVLSHSLLLLHKKEDGIWSTDILKDQKEPKNKTFLRCEAKNYSGRFTCWWLTTISTDLTFSVKSSRGSSDPQGVTCGAATLSAERVRGDNKEYEYSVECQEDSACPAAEESLPIEVMVDAVHKLKYENYTSSFFIRDIIKPDPPKNLQLKPLKNSRQVEVSWEYPDTWSTPHSYFSLTFCVQVQGKSKREKKDRVFTDKTSATVICRKNASISVRAQDRYYSSSWSEWASVPCS

SEQ ID NO: 14 - DNA, 984 bp, Artificial Sequence
  IL-12B nucleotide
atgtgtcaccagcagttggtcatctcttggttttccctggtttttctggcatctcccctcgtggccatatgggaactgaagaaagatgtttatgtcgtagaattggattggtatccggatgcccctggagaaatggtggtcctcacctgtgacacccctgaagaagatggtatcacctggaccttggaccagagcagtgaggtcttaggctctggcaaaaccctgaccatccaagtcaaagagtttggagatgctggccagtacacctgtcacaaaggaggcgaggttctatcccactctctgctgctccttcacaaaaaggaagatggaatttggtccactgatattttaaaggaccagaaagaacccaaaaataagacctttctaagatgcgaggccaagaattattctggacgtttcacctgctggtggctgacgacaatcagtactgatttgacattcagtgtcaaaagcagcagaggctcttctgacccccaaggggtgacgtgcggagctgctacactctctgcagagagagtcagaggggacaacaaggagtatgagtactcagtggagtgccaggaggacagtgcctgcccagctgctgaggagagtctgcccattgaggtcatggtggatgccgttcacaagctcaagtatgaaaactacaccagcagcttcttcatcagggacatcatcaaacctgacccacccaagaacttgcagctgaagccattaaagaattctcggcaggtggaggtcagctgggagtaccctgacacctggagtactccacattcctacttctccctgacattctgcgttcaggtccagggcaagagcaagagagaaaagaaagatagagtcttcacggacaagacctcagccacggtcatctgccgcaaaaatgccagcattagcgtgcgggcccaggaccgctactatagctcatcttggagcgaatgggcatctgtgccctgcagt

SEQ ID NO: 15 - protein, 253 aa, Artificial Sequence
  IL-12A amino acid
MWPPGSASQPPPSPAAATGLHPAARPVSLQCRLSMCPARSLLLVATLVLLDHLSLARNLPVATPDPGMFPCLHHSQNLLRAVSNMLQKARQTLEFYPCTSEEIDHEDITKDKTSTVEACLPLELTKNESCLNSRETSFITNGSCLASRKTSFMMALCLSSIYEDLKMYQVEFKTMNAKLLMDPKRQIFLDQNMLAVIDELMQALNFNSETVPQKSSLEEPDFYKTKIKLCILLHAFRIRAVTIDRVMSYLNAS

SEQ ID NO: 16 - DNA, 759 bp, Artificial Sequence
  IL-12A nucleotide
atgtggccacctggatcagcttctcaaccacctccatcacctgcagctgccacaggtcttcatccagcagctcgacctgtttctcttcagtgtcggctcagcatgtgtccagcgcgcagcctcctccttgtggctaccctggtcctcctggaccacctcagtttggccagaaacctccccgtggccactccagacccaggaatgttcccatgccttcaccactcccaaaacctgctgagggccgtcagcaacatgctccagaaggccagacaaactctagaattttacccttgcacttctgaagagattgatcatgaagatatcacaaaagataaaaccagcacagtggaggcctgtttaccattggaattaaccaagaatgagagttgcctaaattccagagagacctctttcataactaatgggagttgcctggcctccagaaagacctcttttatgatggccctgtgccttagtagtatttatgaagacttgaagatgtaccaggtggagttcaagaccatgaatgcaaagcttctgatggatcctaagaggcagatctttctagatcaaaacatgctggcagttattgatgagctgatgcaggccctgaatttcaacagtgagactgtgccacaaaaatcctcccttgaagaaccggatttttataaaactaaaatcaagctctgcatacttcttcatgctttcagaattcgggcagtgactattgatagagtgatgagctatctgaatgcttcc

SEQ ID NO: 17 - protein, 162 aa, Artificial Sequence
  IL-15 amino acid
MRISKPHLRSISIQCYLCLLLNSHFLTEAGIHVFILGCFSAGLPKTEANWVNVISDLKKIEDLIQSMHIDATLYTESDVHPSCKVTAMKCFLLELQVISLESGDASIHDTVENLIILANNSLSSNGNVTESGCKECEELEEKNIKEFLQSFVHIVQMFINTS

SEQ ID NO: 18 - DNA, 486 bp, Artificial Sequence
  IL-15 nucleotide
atgagaatttcgaaaccacatttgagaagtatttccatccagtgctacttgtgtttacttctaaacagtcattttctaactgaagctggcattcatgtcttcattttgggctgtttcagtgcagggcttcctaaaacagaagccaactgggtgaatgtaataagtgatttgaaaaaaattgaagatcttattcaatctatgcatattgatgctactttatatacggaaagtgatgttcaccccagttgcaaagtaacagcaatgaagtgctttctcttggagttacaagttatttcacttgagtccggagatgcaagtattcatgatacagtagaaaatctgatcatcctagcaaacaacagtttgtcttctaatgggaatgtaacagaatctggatgcaaagaatgtgaggaactggaggaaaaaaatattaaagaatttttgcagagttttgtacatattgtccaaatgttcatcaacacttct

SEQ ID NO: 19 - protein, 162 aa, Artificial Sequence
  IL-21 amino acid
MRSSPGNMERIVICLMVIFLGTLVHKSSSQGQDRHMIRMRQLIDIVDQLKNYVNDLVPEFLPAPEDVETNCEWSAFSCFQKAQLKSANTGNNERIINVSIKKLKRKPPSTNAGRRQKHRLTCPSCDSYEKKPPKEFLERFKSLLQKMIHQHLSSRTHGSEDS

SEQ ID NO: 20 - DNA, 486 bp, Artificial Sequence
  IL-21 nucleotide
atgagatccagtcctggcaacatggagaggattgtcatctgtctgatggtcatcttcttggggacactggtccacaaatcaagctcccaaggtcaagatcgccacatgattagaatgcgtcaacttatagatattgttgatcagctgaaaaattatgtgaatgacttggtccctgaatttctgccagctccagaagatgtagagacaaactgtgagtggtcagctttttcctgctttcagaaggcccaactaaagtcagcaaatacaggaaacaatgaaaggataatcaatgtatcaattaaaaagctgaagaggaaaccaccttccacaaatgcagggagaagacagaaacacagactaacatgcccttcatgtgattcttatgagaaaaaaccacccaaagaattcctagaaagattcaaatcacttctccaaaagatgattcatcagcatctgtcctctagaacacacggaagtgaagattcc

SEQ ID NO: 21 - protein, 218 aa, Artificial Sequence
  IL-37 amino acid
MSFVGENSGVKMGSEDWEKDEPQCCLEDPAGSPLEPGPSLPTMNFVHTSPKVKNLNPKKFSIHDQDHKVLVLDSGNLIAVPDKNYIRPEIFFALASSLSSASAEKGSPILLGVSKGEFCLYCDKDKGQSHPSLQLKKEKLMKLAAQKESARRPFIFYRAQVGSWNMLESAAHPGWFICTSCNCNEPVGVTDKFENRKHIEFSFQPVCKAEMSPSEVSD

SEQ ID NO: 22 - DNA, 654 bp, Artificial Sequence
  IL-37 nucleotide
atgtcctttgtgggggagaactcaggagtgaaaatgggctctgaggactgggaaaaagatgaaccccagtgctgcttagaagacccggctggaagccccctggaaccaggcccaagcctccccaccatgaattttgttcacacaagtccaaaggtgaagaacttaaacccgaagaaattcagcattcatgaccaggatcacaaagtactggtcctggactctgggaatctcatagcagttccagataaaaactacatacgcccagagatcttctttgcattagcctcatccttgagctcagcctctgcggagaaaggaagtccgattctcctgggggtctctaaaggggagttttgtctctactgtgacaaggataaaggacaaagtcatccatcccttcagctgaagaaggagaaactgatgaagctggctgcccaaaaggaatcagcacgccggcccttcatcttttatagggctcaggtgggctcctggaacatgctggagtcggcggctcaccccggatggttcatctgcacctcctgcaattgtaatgagcctgttggggtgacagataaatttgagaacaggaaacacattgaattttcatttcaaccagtttgcaaagctgaaatgagccccagtgaggtcagcgat

SEQ ID NO: 23 - protein, 144 aa, Artificial Sequence
  GM-CSF amino acid
MWLQSLLLLGTVACSISAPARSPSPSTQPWEHVNAIQEARRLLNLSRDTAAEMNETVEVISEMFDLQEPTCLQTRLELYKQGLRGSLTKLKGPLTMMASHYKQHCPPTPETSCATQIITFESFKENLKDFLLVIPFDCWEPVQE

SEQ ID NO: 24 - DNA, 432 bp, Artificial Sequence
  GM-CSF nucleotide
atgtggctgcagagcctgctgctccttggaactgtggcttgttctatctctgcacctgctcgcagtccatctcctagcactcagccatgggagcatgtgaatgccatccaggaggcccggcgtctcctgaacctgagtagagacactgctgctgagatgaatgaaacagtagaagtcatctcagaaatgtttgatcttcaggagccgacatgcctacagacaagactggagctgtacaagcagggactgagaggatctttgacaaagctcaagggccccttgaccatgatggccagccactacaagcagcactgccctccaaccccggaaacttcctgtgcaacccagattatcacctttgaaagtttcaaagagaacctgaaggactttctgcttgtcatcccctttgactgctgggagccagtccaggag

SEQ ID NO: 25 - DNA, 5597 bp, Artificial Sequence
  pDE1
gacggatcgggagatctcccgatcccctatggtgcactctcagtacaatctgctctgatgccgcatagttaagccagtatctgctccctgcttgtgtgttggaggtcgctgagtagtgcgcgagcaaaatttaagctacaacaaggcaaggcttgaccgacaattgcatgaagaatctgcttagggttaggcgttttgcgctgcttcgcgatgtacgggccagatatacgcgttgacattgattattgactagttattaatagtaatcaattacggggtcattagttcatagcccatatatggagttccgcgttacataacttacggtaaatggcccgcctggctgaccgcccaacgacccccgcccattgacgtcaataatgacgtatgttcccatagtaacgccaatagggactttccattgacgtcaatgggtggagtatttacggtaaactgcccacttggcagtacatcaagtgtatcatatgccaagtacgccccctattgacgtcaatgacggtaaatggcccgcctggcattatgcccagtacatgaccttatgggactttcctacttggcagtacatctacgtattagtcatcgctattaccatggtgatgcggttttggcagtacatcaatgggcgtggatagcggtttgactcacggggatttccaagtctccaccccattgacgtcaatgggagtttgttttggcaccaaaatcaacgggactttccaaaatgtcgtaacaactccgccccattgacgcaaatgggcggtaggcgtgtacggtgggaggtctatataagcagagctctctggctaactagagaacccactgcttactggcttatcgaaattaatacgactcactatagggagacccaagctggctagcgtttaaacttaagcttggtaccgagctcggatccactagtccagtgtggtggaattctgcagatatccagcacagtggcggccgctcgagtctagagggcccgtttaaacccgctgatcagcctcgactgtgccttctagttgccagccatctgttgtttgcccctcccccgtgccttccttgaccctggaaggtgccactcccactgtcctttcctaataaaatgaggaaattgcatcgcattgtctgagtaggtgtcattctattctggggggtggggtggggcaggacagcaagggggaggattgggaagacaatagcaggcatgctggggatgcggtgggctctatggcttctgaggcggaaagaaccagctggggctctagggggtatccccacgcgccctgtagcggcgcattaagcgcggcgggtgtggtggttacgcgcagcgtgaccgctacacttgccagcgccctagcgcccgctcctttcgctttcttcccttcctttctcgccacgttcgccggctttccccgtcaagctctaaatcgggggctccctttagggttccgatttagtgctttacggcacctcgaccccaaaaaacttgattagggtgatggttcacgtagtgggccatcgccctgatagacggtttttcgccctttgacgttggagtccacgttctttaatagtggactcttgttccaaactggaacaacactcaaccctatctcggtctattcttttgatttataagggattttgccgatttcggcctattggttaaaaaatgagctgatttaacaaaaatttaacgcgaattaattctgtggaatgtgtgtcagttagggtgtggaaagtccccaggctccccagcaggcagaagtatgcaaagcatgcatctcaattagtcagcaaccaggtgtggaaagtccccaggctccccagcaggcagaagtatgcaaagcatgcatctcaattagtcagcaaccatagtcccgcccctaactccgcccatcccgcccctaactccgcccagttccgcccattctccgccccatggctgactaattttttttatttatgcagaggccgaggccgcctctgcctctgagctattccagaagtagtgaggaggcttttttggaggcctaggcttttgcaaaaagctcccgggagcttgtatatccattttcggatctgatcagcacgtgatgaaaaagcctgaactcaccgcgacgtctgtcgagaagtttctgatcgaaaagttcgacagcgtctccgacctgatgcagctctcggagggcgaagaatctcgtgctttcagcttcgatgtaggagggcgtggatatgtcctgcgggtaaatagctgcgccgatggtttctacaaagatcgttatgtttatcggcactttgcatcggccgcgctcccgattccggaagtgcttgacattggggaattcagcgagagcctgacctattgcatctcccgccgtgcacagggtgtcacgttgcaagacctgcctgaaaccgaactgcccgctgttctgcagccggtcgcggaggccatggatgcgatcgctgcggccgatcttagccagacgagcgggttcggcccattcggaccgcaaggaatcggtcaatacactacatggcgtgatttcatatgcgcgattgctgatccccatgtgtatcactggcaaactgtgatggacgacaccgtcagtgcgtccgtcgcgcaggctctcgatgagctgatgctttgggccgaggactgccccgaagtccggcacctcgtgcacgcggatttcggctccaacaatgtcctgacggacaatggccgcataacagcggtcattgactggagcgaggcgatgttcggggattcccaatacgaggtcgccaacatcttcttctggaggccgtggttggcttgtatggagcagcagacgcgctacttcgagcggaggcatccggagcttgcaggatcgccgcggctccgggcgtatatgctccgcattggtcttgaccaactctatcagagcttggttgacggcaatttcgatgatgcagcttgggcgcagggtcgatgcgacgcaatcgtccgatccggagccgggactgtcgggcgtacacaaatcgcccgcagaagcgcggccgtctggaccgatggctgtgtagaagtactcgccgatagtggaaaccgacgccccagcactcgtccgagggcaaaggaatagcacgtgctacgagatttcgattccaccgccgccttctatgaaaggttgggcttcggaatcgttttccgggacgccggctggatgatcctccagcgcggggatctcatgctggagttcttcgcccaccccaacttgtttattgcagcttataatggttacaaataaagcaatagcatcacaaatttcacaaataaagcatttttttcactgcattctagttgtggtttgtccaaactcatcaatgtatcttatcatgtctgtataccgtcgacctctagctagagcttggcgtaatcatggtcatagctgtttcctgtgtgaaattgttatccgctcacaattccacacaacatacgagccggaagcataaagtgtaaagcctggggtgcctaatgagtgagctaactcacattaattgcgttgcgctcactgcccgctttccagtcgggaaacctgtcgtgccagctgcattaatgaatcggccaacgcgcggggagaggcggtttgcgtattgggcgctcttccgcttcctcgctcactgactcgctgcgctcggtcgttcggctgcggcgagcggtatcagctcactcaaaggcggtaatacggttatccacagaatcaggggataacgcaggaaagaacatgtgagcaaaaggccagcaaaaggccaggaaccgtaaaaaggccgcgttgctggcgtttttccataggctccgcccccctgacgagcatcacaaaaatcgacgctcaagtcagaggtggcgaaacccgacaggactataaagataccaggcgtttccccctggaagctccctcgtgcgctctcctgttccgaccctgccgcttaccggatacctgtccgcctttctcccttcgggaagcgtggcgctttctcatagctcacgctgtaggtatctcagttcggtgtaggtcgttcgctccaagctgggctgtgtgcacgaaccccccgttcagcccgaccgctgcgccttatccggtaactatcgtcttgagtccaacccggtaagacacgacttatcgccactggcagcagccactggtaacaggattagcagagcgaggtatgtaggcggtgctacagagttcttgaagtggtggcctaactacggctacactagaagaacagtatttggtatctgcgctctgctgaagccagttaccttcggaaaaagagttggtagctcttgatccggcaaacaaaccaccgctggtagcggtttttttgtttgcaagcagcagattacgcgcagaaaaaaaggatctcaagaagatcctttgatcttttctacggggtctgacgctcagtggaacgaaaactcacgttaagggattttggtcatgagattatcaaaaaggatcttcacctagatccttttaaattaaaaatgaagttttaaatcaatctaaagtatatatgagtaaacttggtctgacagttaccaatgcttaatcagtgaggcacctatctcagcgatctgtctatttcgttcatccatagttgcctgactccccgtcgtgtagataactacgatacgggagggcttaccatctggccccagtgctgcaatgataccgcgagacccacgctcaccggctccagatttatcagcaataaaccagccagccggaagggccgagcgcagaagtggtcctgcaactttatccgcctccatccagtctattaattgttgccgggaagctagagtaagtagttcgccagttaatagtttgcgcaacgttgttgccattgctacaggcatcgtggtgtcacgctcgtcgtttggtatggcttcattcagctccggttcccaacgatcaaggcgagttacatgatcccccatgttgtgcaaaaaagcggttagctccttcggtcctccgatcgttgtcagaagtaagttggccgcagtgttatcactcatggttatggcagcactgcataattctcttactgtcatgccatccgtaagatgcttttctgtgactggtgagtactcaaccaagtcattctgagaatagtgtatgcggcgaccgagttgctcttgcccggcgtcaatacgggataataccgcgccacatagcagaactttaaaagtgctcatcattggaaaacgttcttcggggcgaaaactctcaaggatcttaccgctgttgagatccagttcgatgtaacccactcgtgcacccaactgatcttcagcatcttttactttcaccagcgtttctgggtgagcaaaaacaggaaggcaaaatgccgcaaaaaagggaataagggcgacacggaaatgttgaatactcatactcttcctttttcaatattattgaagcatttatcagggttattgtctcatgagcggatacatatttgaatgtatttagaaaaataaacaaataggggttccgcgcacatttccccgaaaagtgccacctgacgtc

SEQ ID NO: 26 - DNA, 6641 bp, Artificial Sequence
  pDE1-CYB5R3
gacggatcgggagatctcccgatcccctatggtgcactctcagtacaatctgctctgatgccgcatagttaagccagtatctgctccctgcttgtgtgttggaggtcgctgagtagtgcgcgagcaaaatttaagctacaacaaggcaaggcttgaccgacaattgcatgaagaatctgcttagggttaggcgttttgcgctgcttcgcgatgtacgggccagatatacgcgttgacattgattattgactagttattaatagtaatcaattacggggtcattagttcatagcccatatatggagttccgcgttacataacttacggtaaatggcccgcctggctgaccgcccaacgacccccgcccattgacgtcaataatgacgtatgttcccatagtaacgccaatagggactttccattgacgtcaatgggtggagtatttacggtaaactgcccacttggcagtacatcaagtgtatcatatgccaagtacgccccctattgacgtcaatgacggtaaatggcccgcctggcattatgcccagtacatgaccttatgggactttcctacttggcagtacatctacgtattagtcatcgctattaccatggtgatgcggttttggcagtacatcaatgggcgtggatagcggtttgactcacggggatttccaagtctccaccccattgacgtcaatgggagtttgttttggcaccaaaatcaacgggactttccaaaatgtcgtaacaactccgccccattgacgcaaatgggcggtaggcgtgtacggtgggaggtctatataagcagagctctctggctaactagagaacccactgcttactggcttatcgaaattaatacgactcactatagggagacccaagctggctagcgccaccatgggggcccagctcagcacgttgggccatatggtgctcttcccagtctggttcctgtacagtctgctcatgaagctgttccagcgctccacgccagccatcaccctcgagagcccggacatcaagtatcctctcagactcatcgacagagagatcattagccatgacaccagaaggttcagatttgccctgccttcaccccagcacatcctgggcctccctgtcggccagcacatctacctctcggctcgaattgatggaaacctggtcgtccggccctatacacccatctccagcgatgatgacaagggcttcgtggacctggtcatcaaggtttacttcaaggacacccatcccaagtttcccgctggagggaagatgtctcagtacctggagagcatgcagattggagacaccattgagttccggggccccagtgggctgctggtctaccagggcaaagggaagttcgccatccgacctgacaaaaagtccaaccctatcatcaggacagtgaagtctgtgggcatgatcgcgggagggacaggcatcaccccgatgctgcaggtgatccgcgccatcatgaaggaccctgatgaccacactgtgtgccacctgctctttgccaaccagaccgagaaggacatcctgctgcgacctgagctggaggaactcaggaacaaacattctgcacgcttcaagctctggtacacgctggacagagcccctgaagcctgggactacggccagggcttcgtgaatgaggagatgatccgggaccaccttccacctccagaggaggagcctctggtgctgatgtgtggacctccacctatgatccagtacgcctgccttcccaacctggaccacgtgggccaccccacggagcgctgcttcgtcttcgcctacccttacgacgtcccagactacgctggaagcggagctactaacttcagcctgctgaagcaggctggagacgtggaggagaaccctggacctaagcttggtaccgagctcggatccactagtccagtgtggtggaattctgcagatatccagcacagtggcggccgctcgagtgctggagaacagacaggagactacaaggacgacgatgacaaggcttgatctagagggcccgtttaaacccgctgatcagcctcgactgtgccttctagttgccagccatctgttgtttgcccctcccccgtgccttccttgaccctggaaggtgccactcccactgtcctttcctaataaaatgaggaaattgcatcgcattgtctgagtaggtgtcattctattctggggggtggggtggggcaggacagcaagggggaggattgggaagacaatagcaggcatgctggggatgcggtgggctctatggcttctgaggcggaaagaaccagctggggctctagggggtatccccacgcgccctgtagcggcgcattaagcgcggcgggtgtggtggttacgcgcagcgtgaccgctacacttgccagcgccctagcgcccgctcctttcgctttcttcccttcctttctcgccacgttcgccggctttccccgtcaagctctaaatcgggggctccctttagggttccgatttagtgctttacggcacctcgaccccaaaaaacttgattagggtgatggttcacgtagtgggccatcgccctgatagacggtttttcgccctttgacgttggagtccacgttctttaatagtggactcttgttccaaactggaacaacactcaaccctatctcggtctattcttttgatttataagggattttgccgatttcggcctattggttaaaaaatgagctgatttaacaaaaatttaacgcgaattaattctgtggaatgtgtgtcagttagggtgtggaaagtccccaggctccccagcaggcagaagtatgcaaagcatgcatctcaattagtcagcaaccaggtgtggaaagtccccaggctccccagcaggcagaagtatgcaaagcatgcatctcaattagtcagcaaccatagtcccgcccctaactccgcccatcccgcccctaactccgcccagttccgcccattctccgccccatggctgactaattttttttatttatgcagaggccgaggccgcctctgcctctgagctattccagaagtagtgaggaggcttttttggaggcctaggcttttgcaaaaagctcccgggagcttgtatatccattttcggatctgatcagcacgtgatgaaaaagcctgaactcaccgcgacgtctgtcgagaagtttctgatcgaaaagttcgacagcgtctccgacctgatgcagctctcggagggcgaagaatctcgtgctttcagcttcgatgtaggagggcgtggatatgtcctgcgggtaaatagctgcgccgatggtttctacaaagatcgttatgtttatcggcactttgcatcggccgcgctcccgattccggaagtgcttgacattggggaattcagcgagagcctgacctattgcatctcccgccgtgcacagggtgtcacgttgcaagacctgcctgaaaccgaactgcccgctgttctgcagccggtcgcggaggccatggatgcgatcgctgcggccgatcttagccagacgagcgggttcggcccattcggaccgcaaggaatcggtcaatacactacatggcgtgatttcatatgcgcgattgctgatccccatgtgtatcactggcaaactgtgatggacgacaccgtcagtgcgtccgtcgcgcaggctctcgatgagctgatgctttgggccgaggactgccccgaagtccggcacctcgtgcacgcggatttcggctccaacaatgtcctgacggacaatggccgcataacagcggtcattgactggagcgaggcgatgttcggggattcccaatacgaggtcgccaacatcttcttctggaggccgtggttggcttgtatggagcagcagacgcgctacttcgagcggaggcatccggagcttgcaggatcgccgcggctccgggcgtatatgctccgcattggtcttgaccaactctatcagagcttggttgacggcaatttcgatgatgcagcttgggcgcagggtcgatgcgacgcaatcgtccgatccggagccgggactgtcgggcgtacacaaatcgcccgcagaagcgcggccgtctggaccgatggctgtgtagaagtactcgccgatagtggaaaccgacgccccagcactcgtccgagggcaaaggaatagcacgtgctacgagatttcgattccaccgccgccttctatgaaaggttgggcttcggaatcgttttccgggacgccggctggatgatcctccagcgcggggatctcatgctggagttcttcgcccaccccaacttgtttattgcagcttataatggttacaaataaagcaatagcatcacaaatttcacaaataaagcatttttttcactgcattctagttgtggtttgtccaaactcatcaatgtatcttatcatgtctgtataccgtcgacctctagctagagcttggcgtaatcatggtcatagctgtttcctgtgtgaaattgttatccgctcacaattccacacaacatacgagccggaagcataaagtgtaaagcctggggtgcctaatgagtgagctaactcacattaattgcgttgcgctcactgcccgctttccagtcgggaaacctgtcgtgccagctgcattaatgaatcggccaacgcgcggggagaggcggtttgcgtattgggcgctcttccgcttcctcgctcactgactcgctgcgctcggtcgttcggctgcggcgagcggtatcagctcactcaaaggcggtaatacggttatccacagaatcaggggataacgcaggaaagaacatgtgagcaaaaggccagcaaaaggccaggaaccgtaaaaaggccgcgttgctggcgtttttccataggctccgcccccctgacgagcatcacaaaaatcgacgctcaagtcagaggtggcgaaacccgacaggactataaagataccaggcgtttccccctggaagctccctcgtgcgctctcctgttccgaccctgccgcttaccggatacctgtccgcctttctcccttcgggaagcgtggcgctttctcatagctcacgctgtaggtatctcagttcggtgtaggtcgttcgctccaagctgggctgtgtgcacgaaccccccgttcagcccgaccgctgcgccttatccggtaactatcgtcttgagtccaacccggtaagacacgacttatcgccactggcagcagccactggtaacaggattagcagagcgaggtatgtaggcggtgctacagagttcttgaagtggtggcctaactacggctacactagaagaacagtatttggtatctgcgctctgctgaagccagttaccttcggaaaaagagttggtagctcttgatccggcaaacaaaccaccgctggtagcggtttttttgtttgcaagcagcagattacgcgcagaaaaaaaggatctcaagaagatcctttgatcttttctacggggtctgacgctcagtggaacgaaaactcacgttaagggattttggtcatgagattatcaaaaaggatcttcacctagatccttttaaattaaaaatgaagttttaaatcaatctaaagtatatatgagtaaacttggtctgacagttaccaatgcttaatcagtgaggcacctatctcagcgatctgtctatttcgttcatccatagttgcctgactccccgtcgtgtagataactacgatacgggagggcttaccatctggccccagtgctgcaatgataccgcgagacccacgctcaccggctccagatttatcagcaataaaccagccagccggaagggccgagcgcagaagtggtcctgcaactttatccgcctccatccagtctattaattgttgccgggaagctagagtaagtagttcgccagttaatagtttgcgcaacgttgttgccattgctacaggcatcgtggtgtcacgctcgtcgtttggtatggcttcattcagctccggttcccaacgatcaaggcgagttacatgatcccccatgttgtgcaaaaaagcggttagctccttcggtcctccgatcgttgtcagaagtaagttggccgcagtgttatcactcatggttatggcagcactgcataattctcttactgtcatgccatccgtaagatgcttttctgtgactggtgagtactcaaccaagtcattctgagaatagtgtatgcggcgaccgagttgctcttgcccggcgtcaatacgggataataccgcgccacatagcagaactttaaaagtgctcatcattggaaaacgttcttcggggcgaaaactctcaaggatcttaccgctgttgagatccagttcgatgtaacccactcgtgcacccaactgatcttcagcatcttttactttcaccagcgtttctgggtgagcaaaaacaggaaggcaaaatgccgcaaaaaagggaataagggcgacacggaaatgttgaatactcatactcttcctttttcaatattattgaagcatttatcagggttattgtctcatgagcggatacatatttgaatgtatttagaaaaataaacaaataggggttccgcgcacatttccccgaaaagtgccacctgacgtc

SEQ ID NO: 27 - DNA, 7046 bp, Artificial Sequence
  pDE1-CYB5R3-IL2
gacggatcgggagatctcccgatcccctatggtgcactctcagtacaatctgctctgatgccgcatagttaagccagtatctgctccctgcttgtgtgttggaggtcgctgagtagtgcgcgagcaaaatttaagctacaacaaggcaaggcttgaccgacaattgcatgaagaatctgcttagggttaggcgttttgcgctgcttcgcgatgtacgggccagatatacgcgttgacattgattattgactagttattaatagtaatcaattacggggtcattagttcatagcccatatatggagttccgcgttacataacttacggtaaatggcccgcctggctgaccgcccaacgacccccgcccattgacgtcaataatgacgtatgttcccatagtaacgccaatagggactttccattgacgtcaatgggtggagtatttacggtaaactgcccacttggcagtacatcaagtgtatcatatgccaagtacgccccctattgacgtcaatgacggtaaatggcccgcctggcattatgcccagtacatgaccttatgggactttcctacttggcagtacatctacgtattagtcatcgctattaccatggtgatgcggttttggcagtacatcaatgggcgtggatagcggtttgactcacggggatttccaagtctccaccccattgacgtcaatgggagtttgttttggcaccaaaatcaacgggactttccaaaatgtcgtaacaactccgccccattgacgcaaatgggcggtaggcgtgtacggtgggaggtctatataagcagagctctctggctaactagagaacccactgcttactggcttatcgaaattaatacgactcactatagggagacccaagctggctagcgccaccatgggggcccagctcagcacgttgggccatatggtgctcttcccagtctggttcctgtacagtctgctcatgaagctgttccagcgctccacgccagccatcaccctcgagagcccggacatcaagtatcctctcagactcatcgacagagagatcattagccatgacaccagaaggttcagatttgccctgccttcaccccagcacatcctgggcctccctgtcggccagcacatctacctctcggctcgaattgatggaaacctggtcgtccggccctatacacccatctccagcgatgatgacaagggcttcgtggacctggtcatcaaggtttacttcaaggacacccatcccaagtttcccgctggagggaagatgtctcagtacctggagagcatgcagattggagacaccattgagttccggggccccagtgggctgctggtctaccagggcaaagggaagttcgccatccgacctgacaaaaagtccaaccctatcatcaggacagtgaagtctgtgggcatgatcgcgggagggacaggcatcaccccgatgctgcaggtgatccgcgccatcatgaaggaccctgatgaccacactgtgtgccacctgctctttgccaaccagaccgagaaggacatcctgctgcgacctgagctggaggaactcaggaacaaacattctgcacgcttcaagctctggtacacgctggacagagcccctgaagcctgggactacggccagggcttcgtgaatgaggagatgatccgggaccaccttccacctccagaggaggagcctctggtgctgatgtgtggacctccacctatgatccagtacgcctgccttcccaacctggaccacgtgggccaccccacggagcgctgcttcgtcttcgcctacccttacgacgtcccagactacgctggaagcggagctactaacttcagcctgctgaagcaggctggagacgtggaggagaaccctggacctaagcttggtaccatgtacaggatgcaactcctgtcttgcattgcactaagtcttgcacttgtcacaaacagtgcacctacttcaagttctacaaagaaaacacagctacaactggagcatttactgctggatttacagatgattttgaatggaattaataattacaagaatcccaaactcaccaggatgctcacatttaagttttacatgcccaagaaggccacagaactgaaacatcttcagtgtctagaagaagaactcaaacctctggaggaagtgctaaatttagctcaaagcaaaaactttcacttaagacccagggacttaatcagcaatatcaacgtaatagttctggaactaaagggatctgaaacaacattcatgtgtgaatatgctgatgagacagcaaccattgtagaatttctgaacagatggattaccttttgtcaaagcatcatctcaacactgactggcggccgctcgagtgctggagaacagacaggagactacaaggacgacgatgacaaggcttgatctagagggcccgtttaaacccgctgatcagcctcgactgtgccttctagttgccagccatctgttgtttgcccctcccccgtgccttccttgaccctggaaggtgccactcccactgtcctttcctaataaaatgaggaaattgcatcgcattgtctgagtaggtgtcattctattctggggggtggggtggggcaggacagcaagggggaggattgggaagacaatagcaggcatgctggggatgcggtgggctctatggcttctgaggcggaaagaaccagctggggctctagggggtatccccacgcgccctgtagcggcgcattaagcgcggcgggtgtggtggttacgcgcagcgtgaccgctacacttgccagcgccctagcgcccgctcctttcgctttcttcccttcctttctcgccacgttcgccggctttccccgtcaagctctaaatcgggggctccctttagggttccgatttagtgctttacggcacctcgaccccaaaaaacttgattagggtgatggttcacgtagtgggccatcgccctgatagacggtttttcgccctttgacgttggagtccacgttctttaatagtggactcttgttccaaactggaacaacactcaaccctatctcggtctattcttttgatttataagggattttgccgatttcggcctattggttaaaaaatgagctgatttaacaaaaatttaacgcgaattaattctgtggaatgtgtgtcagttagggtgtggaaagtccccaggctccccagcaggcagaagtatgcaaagcatgcatctcaattagtcagcaaccaggtgtggaaagtccccaggctccccagcaggcagaagtatgcaaagcatgcatctcaattagtcagcaaccatagtcccgcccctaactccgcccatcccgcccctaactccgcccagttccgcccattctccgccccatggctgactaattttttttatttatgcagaggccgaggccgcctctgcctctgagctattccagaagtagtgaggaggcttttttggaggcctaggcttttgcaaaaagctcccgggagcttgtatatccattttcggatctgatcagcacgtgatgaaaaagcctgaactcaccgcgacgtctgtcgagaagtttctgatcgaaaagttcgacagcgtctccgacctgatgcagctctcggagggcgaagaatctcgtgctttcagcttcgatgtaggagggcgtggatatgtcctgcgggtaaatagctgcgccgatggtttctacaaagatcgttatgtttatcggcactttgcatcggccgcgctcccgattccggaagtgcttgacattggggaattcagcgagagcctgacctattgcatctcccgccgtgcacagggtgtcacgttgcaagacctgcctgaaaccgaactgcccgctgttctgcagccggtcgcggaggccatggatgcgatcgctgcggccgatcttagccagacgagcgggttcggcccattcggaccgcaaggaatcggtcaatacactacatggcgtgatttcatatgcgcgattgctgatccccatgtgtatcactggcaaactgtgatggacgacaccgtcagtgcgtccgtcgcgcaggctctcgatgagctgatgctttgggccgaggactgccccgaagtccggcacctcgtgcacgcggatttcggctccaacaatgtcctgacggacaatggccgcataacagcggtcattgactggagcgaggcgatgttcggggattcccaatacgaggtcgccaacatcttcttctggaggccgtggttggcttgtatggagcagcagacgcgctacttcgagcggaggcatccggagcttgcaggatcgccgcggctccgggcgtatatgctccgcattggtcttgaccaactctatcagagcttggttgacggcaatttcgatgatgcagcttgggcgcagggtcgatgcgacgcaatcgtccgatccggagccgggactgtcgggcgtacacaaatcgcccgcagaagcgcggccgtctggaccgatggctgtgtagaagtactcgccgatagtggaaaccgacgccccagcactcgtccgagggcaaaggaatagcacgtgctacgagatttcgattccaccgccgccttctatgaaaggttgggcttcggaatcgttttccgggacgccggctggatgatcctccagcgcggggatctcatgctggagttcttcgcccaccccaacttgtttattgcagcttataatggttacaaataaagcaatagcatcacaaatttcacaaataaagcatttttttcactgcattctagttgtggtttgtccaaactcatcaatgtatcttatcatgtctgtataccgtcgacctctagctagagcttggcgtaatcatggtcatagctgtttcctgtgtgaaattgttatccgctcacaattccacacaacatacgagccggaagcataaagtgtaaagcctggggtgcctaatgagtgagctaactcacattaattgcgttgcgctcactgcccgctttccagtcgggaaacctgtcgtgccagctgcattaatgaatcggccaacgcgcggggagaggcggtttgcgtattgggcgctcttccgcttcctcgctcactgactcgctgcgctcggtcgttcggctgcggcgagcggtatcagctcactcaaaggcggtaatacggttatccacagaatcaggggataacgcaggaaagaacatgtgagcaaaaggccagcaaaaggccaggaaccgtaaaaaggccgcgttgctggcgtttttccataggctccgcccccctgacgagcatcacaaaaatcgacgctcaagtcagaggtggcgaaacccgacaggactataaagataccaggcgtttccccctggaagctccctcgtgcgctctcctgttccgaccctgccgcttaccggatacctgtccgcctttctcccttcgggaagcgtggcgctttctcatagctcacgctgtaggtatctcagttcggtgtaggtcgttcgctccaagctgggctgtgtgcacgaaccccccgttcagcccgaccgctgcgccttatccggtaactatcgtcttgagtccaacccggtaagacacgacttatcgccactggcagcagccactggtaacaggattagcagagcgaggtatgtaggcggtgctacagagttcttgaagtggtggcctaactacggctacactagaagaacagtatttggtatctgcgctctgctgaagccagttaccttcggaaaaagagttggtagctcttgatccggcaaacaaaccaccgctggtagcggtttttttgtttgcaagcagcagattacgcgcagaaaaaaaggatctcaagaagatcctttgatcttttctacggggtctgacgctcagtggaacgaaaactcacgttaagggattttggtcatgagattatcaaaaaggatcttcacctagatccttttaaattaaaaatgaagttttaaatcaatctaaagtatatatgagtaaacttggtctgacagttaccaatgcttaatcagtgaggcacctatctcagcgatctgtctatttcgttcatccatagttgcctgactccccgtcgtgtagataactacgatacgggagggcttaccatctggccccagtgctgcaatgataccgcgagacccacgctcaccggctccagatttatcagcaataaaccagccagccggaagggccgagcgcagaagtggtcctgcaactttatccgcctccatccagtctattaattgttgccgggaagctagagtaagtagttcgccagttaatagtttgcgcaacgttgttgccattgctacaggcatcgtggtgtcacgctcgtcgtttggtatggcttcattcagctccggttcccaacgatcaaggcgagttacatgatcccccatgttgtgcaaaaaagcggttagctccttcggtcctccgatcgttgtcagaagtaagttggccgcagtgttatcactcatggttatggcagcactgcataattctcttactgtcatgccatccgtaagatgcttttctgtgactggtgagtactcaaccaagtcattctgagaatagtgtatgcggcgaccgagttgctcttgcccggcgtcaatacgggataataccgcgccacatagcagaactttaaaagtgctcatcattggaaaacgttcttcggggcgaaaactctcaaggatcttaccgctgttgagatccagttcgatgtaacccactcgtgcacccaactgatcttcagcatcttttactttcaccagcgtttctgggtgagcaaaaacaggaaggcaaaatgccgcaaaaaagggaataagggcgacacggaaatgttgaatactcatactcttcctttttcaatattattgaagcatttatcagggttattgtctcatgagcggatacatatttgaatgtatttagaaaaataaacaaataggggttccgcgcacatttccccgaaaagtgccacctgacgtc

SEQ ID NO: 28 - DNA, 7118 bp, Artificial Sequence
  pDE1-CYB5R3-IL7
gacggatcgggagatctcccgatcccctatggtgcactctcagtacaatctgctctgatgccgcatagttaagccagtatctgctccctgcttgtgtgttggaggtcgctgagtagtgcgcgagcaaaatttaagctacaacaaggcaaggcttgaccgacaattgcatgaagaatctgcttagggttaggcgttttgcgctgcttcgcgatgtacgggccagatatacgcgttgacattgattattgactagttattaatagtaatcaattacggggtcattagttcatagcccatatatggagttccgcgttacataacttacggtaaatggcccgcctggctgaccgcccaacgacccccgcccattgacgtcaataatgacgtatgttcccatagtaacgccaatagggactttccattgacgtcaatgggtggagtatttacggtaaactgcccacttggcagtacatcaagtgtatcatatgccaagtacgccccctattgacgtcaatgacggtaaatggcccgcctggcattatgcccagtacatgaccttatgggactttcctacttggcagtacatctacgtattagtcatcgctattaccatggtgatgcggttttggcagtacatcaatgggcgtggatagcggtttgactcacggggatttccaagtctccaccccattgacgtcaatgggagtttgttttggcaccaaaatcaacgggactttccaaaatgtcgtaacaactccgccccattgacgcaaatgggcggtaggcgtgtacggtgggaggtctatataagcagagctctctggctaactagagaacccactgcttactggcttatcgaaattaatacgactcactatagggagacccaagctggctagcgccaccatgggggcccagctcagcacgttgggccatatggtgctcttcccagtctggttcctgtacagtctgctcatgaagctgttccagcgctccacgccagccatcaccctcgagagcccggacatcaagtatcctctcagactcatcgacagagagatcattagccatgacaccagaaggttcagatttgccctgccttcaccccagcacatcctgggcctccctgtcggccagcacatctacctctcggctcgaattgatggaaacctggtcgtccggccctatacacccatctccagcgatgatgacaagggcttcgtggacctggtcatcaaggtttacttcaaggacacccatcccaagtttcccgctggagggaagatgtctcagtacctggagagcatgcagattggagacaccattgagttccggggccccagtgggctgctggtctaccagggcaaagggaagttcgccatccgacctgacaaaaagtccaaccctatcatcaggacagtgaagtctgtgggcatgatcgcgggagggacaggcatcaccccgatgctgcaggtgatccgcgccatcatgaaggaccctgatgaccacactgtgtgccacctgctctttgccaaccagaccgagaaggacatcctgctgcgacctgagctggaggaactcaggaacaaacattctgcacgcttcaagctctggtacacgctggacagagcccctgaagcctgggactacggccagggcttcgtgaatgaggagatgatccgggaccaccttccacctccagaggaggagcctctggtgctgatgtgtggacctccacctatgatccagtacgcctgccttcccaacctggaccacgtgggccaccccacggagcgctgcttcgtcttcgcctacccttacgacgtcccagactacgctggaagcggagctactaacttcagcctgctgaagcaggctggagacgtggaggagaaccctggacctaagcttggtaccatgttccatgtttcttttaggtatatctttggacttcctcccctgatccttgttctgttgccagtagcatcatctgattgtgatattgaaggtaaagatggcaaacaatatgagagtgttctaatggtcagcatcgatcaattattggacagcatgaaagaaattggtagcaattgcctgaataatgaatttaacttttttaaaagacatatctgtgatgctaataaggaaggtatgtttttattccgtgctgctcgcaagttgaggcaatttcttaaaatgaatagcactggtgattttgatctccacttattaaaagtttcagaaggcacaacaatactgttgaactgcactggccaggttaaaggaagaaaaccagctgccctgggtgaagcccaaccaacaaagagtttggaagaaaataaatctttaaaggaacagaaaaaactgaatgacttgtgtttcctaaagagactattacaagagataaaaacttgttggaataaaattttgatgggcactaaagaacacggcggccgctcgagtgctggagaacagacaggagactacaaggacgacgatgacaaggcttgatctagagggcccgtttaaacccgctgatcagcctcgactgtgccttctagttgccagccatctgttgtttgcccctcccccgtgccttccttgaccctggaaggtgccactcccactgtcctttcctaataaaatgaggaaattgcatcgcattgtctgagtaggtgtcattctattctggggggtggggtggggcaggacagcaagggggaggattgggaagacaatagcaggcatgctggggatgcggtgggctctatggcttctgaggcggaaagaaccagctggggctctagggggtatccccacgcgccctgtagcggcgcattaagcgcggcgggtgtggtggttacgcgcagcgtgaccgctacacttgccagcgccctagcgcccgctcctttcgctttcttcccttcctttctcgccacgttcgccggctttccccgtcaagctctaaatcgggggctccctttagggttccgatttagtgctttacggcacctcgaccccaaaaaacttgattagggtgatggttcacgtagtgggccatcgccctgatagacggtttttcgccctttgacgttggagtccacgttctttaatagtggactcttgttccaaactggaacaacactcaaccctatctcggtctattcttttgatttataagggattttgccgatttcggcctattggttaaaaaatgagctgatttaacaaaaatttaacgcgaattaattctgtggaatgtgtgtcagttagggtgtggaaagtccccaggctccccagcaggcagaagtatgcaaagcatgcatctcaattagtcagcaaccaggtgtggaaagtccccaggctccccagcaggcagaagtatgcaaagcatgcatctcaattagtcagcaaccatagtcccgcccctaactccgcccatcccgcccctaactccgcccagttccgcccattctccgccccatggctgactaattttttttatttatgcagaggccgaggccgcctctgcctctgagctattccagaagtagtgaggaggcttttttggaggcctaggcttttgcaaaaagctcccgggagcttgtatatccattttcggatctgatcagcacgtgatgaaaaagcctgaactcaccgcgacgtctgtcgagaagtttctgatcgaaaagttcgacagcgtctccgacctgatgcagctctcggagggcgaagaatctcgtgctttcagcttcgatgtaggagggcgtggatatgtcctgcgggtaaatagctgcgccgatggtttctacaaagatcgttatgtttatcggcactttgcatcggccgcgctcccgattccggaagtgcttgacattggggaattcagcgagagcctgacctattgcatctcccgccgtgcacagggtgtcacgttgcaagacctgcctgaaaccgaactgcccgctgttctgcagccggtcgcggaggccatggatgcgatcgctgcggccgatcttagccagacgagcgggttcggcccattcggaccgcaaggaatcggtcaatacactacatggcgtgatttcatatgcgcgattgctgatccccatgtgtatcactggcaaactgtgatggacgacaccgtcagtgcgtccgtcgcgcaggctctcgatgagctgatgctttgggccgaggactgccccgaagtccggcacctcgtgcacgcggatttcggctccaacaatgtcctgacggacaatggccgcataacagcggtcattgactggagcgaggcgatgttcggggattcccaatacgaggtcgccaacatcttcttctggaggccgtggttggcttgtatggagcagcagacgcgctacttcgagcggaggcatccggagcttgcaggatcgccgcggctccgggcgtatatgctccgcattggtcttgaccaactctatcagagcttggttgacggcaatttcgatgatgcagcttgggcgcagggtcgatgcgacgcaatcgtccgatccggagccgggactgtcgggcgtacacaaatcgcccgcagaagcgcggccgtctggaccgatggctgtgtagaagtactcgccgatagtggaaaccgacgccccagcactcgtccgagggcaaaggaatagcacgtgctacgagatttcgattccaccgccgccttctatgaaaggttgggcttcggaatcgttttccgggacgccggctggatgatcctccagcgcggggatctcatgctggagttcttcgcccaccccaacttgtttattgcagcttataatggttacaaataaagcaatagcatcacaaatttcacaaataaagcatttttttcactgcattctagttgtggtttgtccaaactcatcaatgtatcttatcatgtctgtataccgtcgacctctagctagagcttggcgtaatcatggtcatagctgtttcctgtgtgaaattgttatccgctcacaattccacacaacatacgagccggaagcataaagtgtaaagcctggggtgcctaatgagtgagctaactcacattaattgcgttgcgctcactgcccgctttccagtcgggaaacctgtcgtgccagctgcattaatgaatcggccaacgcgcggggagaggcggtttgcgtattgggcgctcttccgcttcctcgctcactgactcgctgcgctcggtcgttcggctgcggcgagcggtatcagctcactcaaaggcggtaatacggttatccacagaatcaggggataacgcaggaaagaacatgtgagcaaaaggccagcaaaaggccaggaaccgtaaaaaggccgcgttgctggcgtttttccataggctccgcccccctgacgagcatcacaaaaatcgacgctcaagtcagaggtggcgaaacccgacaggactataaagataccaggcgtttccccctggaagctccctcgtgcgctctcctgttccgaccctgccgcttaccggatacctgtccgcctttctcccttcgggaagcgtggcgctttctcatagctcacgctgtaggtatctcagttcggtgtaggtcgttcgctccaagctgggctgtgtgcacgaaccccccgttcagcccgaccgctgcgccttatccggtaactatcgtcttgagtccaacccggtaagacacgacttatcgccactggcagcagccactggtaacaggattagcagagcgaggtatgtaggcggtgctacagagttcttgaagtggtggcctaactacggctacactagaagaacagtatttggtatctgcgctctgctgaagccagttaccttcggaaaaagagttggtagctcttgatccggcaaacaaaccaccgctggtagcggtttttttgtttgcaagcagcagattacgcgcagaaaaaaaggatctcaagaagatcctttgatcttttctacggggtctgacgctcagtggaacgaaaactcacgttaagggattttggtcatgagattatcaaaaaggatcttcacctagatccttttaaattaaaaatgaagttttaaatcaatctaaagtatatatgagtaaacttggtctgacagttaccaatgcttaatcagtgaggcacctatctcagcgatctgtctatttcgttcatccatagttgcctgactccccgtcgtgtagataactacgatacgggagggcttaccatctggccccagtgctgcaatgataccgcgagacccacgctcaccggctccagatttatcagcaataaaccagccagccggaagggccgagcgcagaagtggtcctgcaactttatccgcctccatccagtctattaattgttgccgggaagctagagtaagtagttcgccagttaatagtttgcgcaacgttgttgccattgctacaggcatcgtggtgtcacgctcgtcgtttggtatggcttcattcagctccggttcccaacgatcaaggcgagttacatgatcccccatgttgtgcaaaaaagcggttagctccttcggtcctccgatcgttgtcagaagtaagttggccgcagtgttatcactcatggttatggcagcactgcataattctcttactgtcatgccatccgtaagatgcttttctgtgactggtgagtactcaaccaagtcattctgagaatagtgtatgcggcgaccgagttgctcttgcccggcgtcaatacgggataataccgcgccacatagcagaactttaaaagtgctcatcattggaaaacgttcttcggggcgaaaactctcaaggatcttaccgctgttgagatccagttcgatgtaacccactcgtgcacccaactgatcttcagcatcttttactttcaccagcgtttctgggtgagcaaaaacaggaaggcaaaatgccgcaaaaaagggaataagggcgacacggaaatgttgaatactcatactcttcctttttcaatattattgaagcatttatcagggttattgtctcatgagcggatacatatttgaatgtatttagaaaaataaacaaataggggttccgcgcacatttccccgaaaagtgccacctgacgtc

SEQ ID NO: 29 - DNA, 8225 bp, Artificial Sequence
  pDE1-CYB5R3-IL12(p70)
gacggatcgggagatctcccgatcccctatggtgcactctcagtacaatctgctctgatgccgcatagttaagccagtatctgctccctgcttgtgtgttggaggtcgctgagtagtgcgcgagcaaaatttaagctacaacaaggcaaggcttgaccgacaattgcatgaagaatctgcttagggttaggcgttttgcgctgcttcgcgatgtacgggccagatatacgcgttgacattgattattgactagttattaatagtaatcaattacggggtcattagttcatagcccatatatggagttccgcgttacataacttacggtaaatggcccgcctggctgaccgcccaacgacccccgcccattgacgtcaataatgacgtatgttcccatagtaacgccaatagggactttccattgacgtcaatgggtggagtatttacggtaaactgcccacttggcagtacatcaagtgtatcatatgccaagtacgccccctattgacgtcaatgacggtaaatggcccgcctggcattatgcccagtacatgaccttatgggactttcctacttggcagtacatctacgtattagtcatcgctattaccatggtgatgcggttttggcagtacatcaatgggcgtggatagcggtttgactcacggggatttccaagtctccaccccattgacgtcaatgggagtttgttttggcaccaaaatcaacgggactttccaaaatgtcgtaacaactccgccccattgacgcaaatgggcggtaggcgtgtacggtgggaggtctatataagcagagctctctggctaactagagaacccactgcttactggcttatcgaaattaatacgactcactatagggagacccaagctggctagcgccaccatgggggcccagctcagcacgttgggccatatggtgctcttcccagtctggttcctgtacagtctgctcatgaagctgttccagcgctccacgccagccatcaccctcgagagcccggacatcaagtatcctctcagactcatcgacagagagatcattagccatgacaccagaaggttcagatttgccctgccttcaccccagcacatcctgggcctccctgtcggccagcacatctacctctcggctcgaattgatggaaacctggtcgtccggccctatacacccatctccagcgatgatgacaagggcttcgtggacctggtcatcaaggtttacttcaaggacacccatcccaagtttcccgctggagggaagatgtctcagtacctggagagcatgcagattggagacaccattgagttccggggccccagtgggctgctggtctaccagggcaaagggaagttcgccatccgacctgacaaaaagtccaaccctatcatcaggacagtgaagtctgtgggcatgatcgcgggagggacaggcatcaccccgatgctgcaggtgatccgcgccatcatgaaggaccctgatgaccacactgtgtgccacctgctctttgccaaccagaccgagaaggacatcctgctgcgacctgagctggaggaactcaggaacaaacattctgcacgcttcaagctctggtacacgctggacagagcccctgaagcctgggactacggccagggcttcgtgaatgaggagatgatccgggaccaccttccacctccagaggaggagcctctggtgctgatgtgtggacctccacctatgatccagtacgcctgccttcccaacctggaccacgtgggccaccccacggagcgctgcttcgtcttcgcctacccttacgacgtcccagactacgctggaagcggagctactaacttcagcctgctgaagcaggctggagacgtggaggagaaccctggacctaagcttggtaccatgtgtcaccagcagttggtcatctcttggttttccctggtttttctggcatctcccctcgtggccatatgggaactgaagaaagatgtttatgtcgtagaattggattggtatccggatgcccctggagaaatggtggtcctcacctgtgacacccctgaagaagatggtatcacctggaccttggaccagagcagtgaggtcttaggctctggcaaaaccctgaccatccaagtcaaagagtttggagatgctggccagtacacctgtcacaaaggaggcgaggttctatcccactctctgctgctccttcacaaaaaggaagatggaatttggtccactgatattttaaaggaccagaaagaacccaaaaataagacctttctaagatgcgaggccaagaattattctggacgtttcacctgctggtggctgacgacaatcagtactgatttgacattcagtgtcaaaagcagcagaggctcttctgacccccaaggggtgacgtgcggagctgctacactctctgcagagagagtcagaggggacaacaaggagtatgagtactcagtggagtgccaggaggacagtgcctgcccagctgctgaggagagtctgcccattgaggtcatggtggatgccgttcacaagctcaagtatgaaaactacaccagcagcttcttcatcagggacatcatcaaacctgacccacccaagaacttgcagctgaagccattaaagaattctcggcaggtggaggtcagctgggagtaccctgacacctggagtactccacattcctacttctccctgacattctgcgttcaggtccagggcaagagcaagagagaaaagaaagatagagtcttcacggacaagacctcagccacggtcatctgccgcaaaaatgccagcattagcgtgcgggcccaggaccgctactatagctcatcttggagcgaatgggcatctgtgccctgcagtaagggtggatctgaaggaggttcaggatctgaagctggtggagagtcctctggaggacgtgaaagaaacctccccgtggccactccagacccaggaatgttcccatgccttcaccactcccaaaacctgctgagggccgtcagcaacatgctccagaaggccagacaaactctagaattttacccttgcacttctgaagagattgatcatgaagatatcacaaaagataaaaccagcacagtggaggcctgtttaccattggaattaaccaagaatgagagttgcctaaattccagagagacctctttcataactaatgggagttgcctggcctccagaaagacctcttttatgatggccctgtgccttagtagtatttatgaagacttgaagatgtaccaggtggagttcaagaccatgaatgcaaagcttctgatggatcctaagaggcagatctttctagatcaaaacatgctggcagttattgatgagctgatgcaggccctgaatttcaacagtgagactgtgccacaaaaatcctcccttgaagaaccggatttttataaaactaaaatcaagctctgcatacttcttcatgctttcagaattcgggcagtgactattgatagagtgatgagctatctgaatgcttccggcggccgctcgagtgctggagaacagacaggagactacaaggacgacgatgacaaggcttgatctagagggcccgtttaaacccgctgatcagcctcgactgtgccttctagttgccagccatctgttgtttgcccctcccccgtgccttccttgaccctggaaggtgccactcccactgtcctttcctaataaaatgaggaaattgcatcgcattgtctgagtaggtgtcattctattctggggggtggggtggggcaggacagcaagggggaggattgggaagacaatagcaggcatgctggggatgcggtgggctctatggcttctgaggcggaaagaaccagctggggctctagggggtatccccacgcgccctgtagcggcgcattaagcgcggcgggtgtggtggttacgcgcagcgtgaccgctacacttgccagcgccctagcgcccgctcctttcgctttcttcccttcctttctcgccacgttcgccggctttccccgtcaagctctaaatcgggggctccctttagggttccgatttagtgctttacggcacctcgaccccaaaaaacttgattagggtgatggttcacgtagtgggccatcgccctgatagacggtttttcgccctttgacgttggagtccacgttctttaatagtggactcttgttccaaactggaacaacactcaaccctatctcggtctattcttttgatttataagggattttgccgatttcggcctattggttaaaaaatgagctgatttaacaaaaatttaacgcgaattaattctgtggaatgtgtgtcagttagggtgtggaaagtccccaggctccccagcaggcagaagtatgcaaagcatgcatctcaattagtcagcaaccaggtgtggaaagtccccaggctccccagcaggcagaagtatgcaaagcatgcatctcaattagtcagcaaccatagtcccgcccctaactccgcccatcccgcccctaactccgcccagttccgcccattctccgccccatggctgactaattttttttatttatgcagaggccgaggccgcctctgcctctgagctattccagaagtagtgaggaggcttttttggaggcctaggcttttgcaaaaagctcccgggagcttgtatatccattttcggatctgatcagcacgtgatgaaaaagcctgaactcaccgcgacgtctgtcgagaagtttctgatcgaaaagttcgacagcgtctccgacctgatgcagctctcggagggcgaagaatctcgtgctttcagcttcgatgtaggagggcgtggatatgtcctgcgggtaaatagctgcgccgatggtttctacaaagatcgttatgtttatcggcactttgcatcggccgcgctcccgattccggaagtgcttgacattggggaattcagcgagagcctgacctattgcatctcccgccgtgcacagggtgtcacgttgcaagacctgcctgaaaccgaactgcccgctgttctgcagccggtcgcggaggccatggatgcgatcgctgcggccgatcttagccagacgagcgggttcggcccattcggaccgcaaggaatcggtcaatacactacatggcgtgatttcatatgcgcgattgctgatccccatgtgtatcactggcaaactgtgatggacgacaccgtcagtgcgtccgtcgcgcaggctctcgatgagctgatgctttgggccgaggactgccccgaagtccggcacctcgtgcacgcggatttcggctccaacaatgtcctgacggacaatggccgcataacagcggtcattgactggagcgaggcgatgttcggggattcccaatacgaggtcgccaacatcttcttctggaggccgtggttggcttgtatggagcagcagacgcgctacttcgagcggaggcatccggagcttgcaggatcgccgcggctccgggcgtatatgctccgcattggtcttgaccaactctatcagagcttggttgacggcaatttcgatgatgcagcttgggcgcagggtcgatgcgacgcaatcgtccgatccggagccgggactgtcgggcgtacacaaatcgcccgcagaagcgcggccgtctggaccgatggctgtgtagaagtactcgccgatagtggaaaccgacgccccagcactcgtccgagggcaaaggaatagcacgtgctacgagatttcgattccaccgccgccttctatgaaaggttgggcttcggaatcgttttccgggacgccggctggatgatcctccagcgcggggatctcatgctggagttcttcgcccaccccaacttgtttattgcagcttataatggttacaaataaagcaatagcatcacaaatttcacaaataaagcatttttttcactgcattctagttgtggtttgtccaaactcatcaatgtatcttatcatgtctgtataccgtcgacctctagctagagcttggcgtaatcatggtcatagctgtttcctgtgtgaaattgttatccgctcacaattccacacaacatacgagccggaagcataaagtgtaaagcctggggtgcctaatgagtgagctaactcacattaattgcgttgcgctcactgcccgctttccagtcgggaaacctgtcgtgccagctgcattaatgaatcggccaacgcgcggggagaggcggtttgcgtattgggcgctcttccgcttcctcgctcactgactcgctgcgctcggtcgttcggctgcggcgagcggtatcagctcactcaaaggcggtaatacggttatccacagaatcaggggataacgcaggaaagaacatgtgagcaaaaggccagcaaaaggccaggaaccgtaaaaaggccgcgttgctggcgtttttccataggctccgcccccctgacgagcatcacaaaaatcgacgctcaagtcagaggtggcgaaacccgacaggactataaagataccaggcgtttccccctggaagctccctcgtgcgctctcctgttccgaccctgccgcttaccggatacctgtccgcctttctcccttcgggaagcgtggcgctttctcatagctcacgctgtaggtatctcagttcggtgtaggtcgttcgctccaagctgggctgtgtgcacgaaccccccgttcagcccgaccgctgcgccttatccggtaactatcgtcttgagtccaacccggtaagacacgacttatcgccactggcagcagccactggtaacaggattagcagagcgaggtatgtaggcggtgctacagagttcttgaagtggtggcctaactacggctacactagaagaacagtatttggtatctgcgctctgctgaagccagttaccttcggaaaaagagttggtagctcttgatccggcaaacaaaccaccgctggtagcggtttttttgtttgcaagcagcagattacgcgcagaaaaaaaggatctcaagaagatcctttgatcttttctacggggtctgacgctcagtggaacgaaaactcacgttaagggattttggtcatgagattatcaaaaaggatcttcacctagatccttttaaattaaaaatgaagttttaaatcaatctaaagtatatatgagtaaacttggtctgacagttaccaatgcttaatcagtgaggcacctatctcagcgatctgtctatttcgttcatccatagttgcctgactccccgtcgtgtagataactacgatacgggagggcttaccatctggccccagtgctgcaatgataccgcgagacccacgctcaccggctccagatttatcagcaataaaccagccagccggaagggccgagcgcagaagtggtcctgcaactttatccgcctccatccagtctattaattgttgccgggaagctagagtaagtagttcgccagttaatagtttgcgcaacgttgttgccattgctacaggcatcgtggtgtcacgctcgtcgtttggtatggcttcattcagctccggttcccaacgatcaaggcgagttacatgatcccccatgttgtgcaaaaaagcggttagctccttcggtcctccgatcgttgtcagaagtaagttggccgcagtgttatcactcatggttatggcagcactgcataattctcttactgtcatgccatccgtaagatgcttttctgtgactggtgagtactcaaccaagtcattctgagaatagtgtatgcggcgaccgagttgctcttgcccggcgtcaatacgggataataccgcgccacatagcagaactttaaaagtgctcatcattggaaaacgttcttcggggcgaaaactctcaaggatcttaccgctgttgagatccagttcgatgtaacccactcgtgcacccaactgatcttcagcatcttttactttcaccagcgtttctgggtgagcaaaaacaggaaggcaaaatgccgcaaaaaagggaataagggcgacacggaaatgttgaatactcatactcttcctttttcaatattattgaagcatttatcagggttattgtctcatgagcggatacatatttgaatgtatttagaaaaataaacaaataggggttccgcgcacatttccccgaaaagtgccacctgacgtc

SEQ ID NO: 30 - DNA, 7346 bp, Artificial Sequence
  pDE1-CYB5R3-IL12A
gacggatcgggagatctcccgatcccctatggtgcactctcagtacaatctgctctgatgccgcatagttaagccagtatctgctccctgcttgtgtgttggaggtcgctgagtagtgcgcgagcaaaatttaagctacaacaaggcaaggcttgaccgacaattgcatgaagaatctgcttagggttaggcgttttgcgctgcttcgcgatgtacgggccagatatacgcgttgacattgattattgactagttattaatagtaatcaattacggggtcattagttcatagcccatatatggagttccgcgttacataacttacggtaaatggcccgcctggctgaccgcccaacgacccccgcccattgacgtcaataatgacgtatgttcccatagtaacgccaatagggactttccattgacgtcaatgggtggagtatttacggtaaactgcccacttggcagtacatcaagtgtatcatatgccaagtacgccccctattgacgtcaatgacggtaaatggcccgcctggcattatgcccagtacatgaccttatgggactttcctacttggcagtacatctacgtattagtcatcgctattaccatggtgatgcggttttggcagtacatcaatgggcgtggatagcggtttgactcacggggatttccaagtctccaccccattgacgtcaatgggagtttgttttggcaccaaaatcaacgggactttccaaaatgtcgtaacaactccgccccattgacgcaaatgggcggtaggcgtgtacggtgggaggtctatataagcagagctctctggctaactagagaacccactgcttactggcttatcgaaattaatacgactcactatagggagacccaagctggctagcgccaccatgggggcccagctcagcacgttgggccatatggtgctcttcccagtctggttcctgtacagtctgctcatgaagctgttccagcgctccacgccagccatcaccctcgagagcccggacatcaagtatcctctcagactcatcgacagagagatcattagccatgacaccagaaggttcagatttgccctgccttcaccccagcacatcctgggcctccctgtcggccagcacatctacctctcggctcgaattgatggaaacctggtcgtccggccctatacacccatctccagcgatgatgacaagggcttcgtggacctggtcatcaaggtttacttcaaggacacccatcccaagtttcccgctggagggaagatgtctcagtacctggagagcatgcagattggagacaccattgagttccggggccccagtgggctgctggtctaccagggcaaagggaagttcgccatccgacctgacaaaaagtccaaccctatcatcaggacagtgaagtctgtgggcatgatcgcgggagggacaggcatcaccccgatgctgcaggtgatccgcgccatcatgaaggaccctgatgaccacactgtgtgccacctgctctttgccaaccagaccgagaaggacatcctgctgcgacctgagctggaggaactcaggaacaaacattctgcacgcttcaagctctggtacacgctggacagagcccctgaagcctgggactacggccagggcttcgtgaatgaggagatgatccgggaccaccttccacctccagaggaggagcctctggtgctgatgtgtggacctccacctatgatccagtacgcctgccttcccaacctggaccacgtgggccaccccacggagcgctgcttcgtcttcgcctacccttacgacgtcccagactacgctggaagcggagctactaacttcagcctgctgaagcaggctggagacgtggaggagaaccctggacctaagcttggtaccatgtggccacctggatcagcttctcaaccacctccatcacctgcagctgccacaggtcttcatccagcagctcgacctgtttctcttcagtgtcggctcagcatgtgtccagcgcgcagcctcctccttgtggctaccctggtcctcctggaccacctcagtttggccagaaacctccccgtggccactccagacccaggaatgttcccatgccttcaccactcccaaaacctgctgagggccgtcagcaacatgctccagaaggccagacaaactctagaattttacccttgcacttctgaagagattgatcatgaagatatcacaaaagataaaaccagcacagtggaggcctgtttaccattggaattaaccaagaatgagagttgcctaaattccagagagacctctttcataactaatgggagttgcctggcctccagaaagacctcttttatgatggccctgtgccttagtagtatttatgaagacttgaagatgtaccaggtggagttcaagaccatgaatgcaaagcttctgatggatcctaagaggcagatctttctagatcaaaacatgctggcagttattgatgagctgatgcaggccctgaatttcaacagtgagactgtgccacaaaaatcctcccttgaagaaccggatttttataaaactaaaatcaagctctgcatacttcttcatgctttcagaattcgggcagtgactattgatagagtgatgagctatctgaatgcttccggcggccgctcgagtgctggagaacagacaggagactacaaggacgacgatgacaaggcttgatctagagggcccgtttaaacccgctgatcagcctcgactgtgccttctagttgccagccatctgttgtttgcccctcccccgtgccttccttgaccctggaaggtgccactcccactgtcctttcctaataaaatgaggaaattgcatcgcattgtctgagtaggtgtcattctattctggggggtggggtggggcaggacagcaagggggaggattgggaagacaatagcaggcatgctggggatgcggtgggctctatggcttctgaggcggaaagaaccagctggggctctagggggtatccccacgcgccctgtagcggcgcattaagcgcggcgggtgtggtggttacgcgcagcgtgaccgctacacttgccagcgccctagcgcccgctcctttcgctttcttcccttcctttctcgccacgttcgccggctttccccgtcaagctctaaatcgggggctccctttagggttccgatttagtgctttacggcacctcgaccccaaaaaacttgattagggtgatggttcacgtagtgggccatcgccctgatagacggtttttcgccctttgacgttggagtccacgttctttaatagtggactcttgttccaaactggaacaacactcaaccctatctcggtctattcttttgatttataagggattttgccgatttcggcctattggttaaaaaatgagctgatttaacaaaaatttaacgcgaattaattctgtggaatgtgtgtcagttagggtgtggaaagtccccaggctccccagcaggcagaagtatgcaaagcatgcatctcaattagtcagcaaccaggtgtggaaagtccccaggctccccagcaggcagaagtatgcaaagcatgcatctcaattagtcagcaaccatagtcccgcccctaactccgcccatcccgcccctaactccgcccagttccgcccattctccgccccatggctgactaattttttttatttatgcagaggccgaggccgcctctgcctctgagctattccagaagtagtgaggaggcttttttggaggcctaggcttttgcaaaaagctcccgggagcttgtatatccattttcggatctgatcagcacgtgatgaaaaagcctgaactcaccgcgacgtctgtcgagaagtttctgatcgaaaagttcgacagcgtctccgacctgatgcagctctcggagggcgaagaatctcgtgctttcagcttcgatgtaggagggcgtggatatgtcctgcgggtaaatagctgcgccgatggtttctacaaagatcgttatgtttatcggcactttgcatcggccgcgctcccgattccggaagtgcttgacattggggaattcagcgagagcctgacctattgcatctcccgccgtgcacagggtgtcacgttgcaagacctgcctgaaaccgaactgcccgctgttctgcagccggtcgcggaggccatggatgcgatcgctgcggccgatcttagccagacgagcgggttcggcccattcggaccgcaaggaatcggtcaatacactacatggcgtgatttcatatgcgcgattgctgatccccatgtgtatcactggcaaactgtgatggacgacaccgtcagtgcgtccgtcgcgcaggctctcgatgagctgatgctttgggccgaggactgccccgaagtccggcacctcgtgcacgcggatttcggctccaacaatgtcctgacggacaatggccgcataacagcggtcattgactggagcgaggcgatgttcggggattcccaatacgaggtcgccaacatcttcttctggaggccgtggttggcttgtatggagcagcagacgcgctacttcgagcggaggcatccggagcttgcaggatcgccgcggctccgggcgtatatgctccgcattggtcttgaccaactctatcagagcttggttgacggcaatttcgatgatgcagcttgggcgcagggtcgatgcgacgcaatcgtccgatccggagccgggactgtcgggcgtacacaaatcgcccgcagaagcgcggccgtctggaccgatggctgtgtagaagtactcgccgatagtggaaaccgacgccccagcactcgtccgagggcaaaggaatagcacgtgctacgagatttcgattccaccgccgccttctatgaaaggttgggcttcggaatcgttttccgggacgccggctggatgatcctccagcgcggggatctcatgctggagttcttcgcccaccccaacttgtttattgcagcttataatggttacaaataaagcaatagcatcacaaatttcacaaataaagcatttttttcactgcattctagttgtggtttgtccaaactcatcaatgtatcttatcatgtctgtataccgtcgacctctagctagagcttggcgtaatcatggtcatagctgtttcctgtgtgaaattgttatccgctcacaattccacacaacatacgagccggaagcataaagtgtaaagcctggggtgcctaatgagtgagctaactcacattaattgcgttgcgctcactgcccgctttccagtcgggaaacctgtcgtgccagctgcattaatgaatcggccaacgcgcggggagaggcggtttgcgtattgggcgctcttccgcttcctcgctcactgactcgctgcgctcggtcgttcggctgcggcgagcggtatcagctcactcaaaggcggtaatacggttatccacagaatcaggggataacgcaggaaagaacatgtgagcaaaaggccagcaaaaggccaggaaccgtaaaaaggccgcgttgctggcgtttttccataggctccgcccccctgacgagcatcacaaaaatcgacgctcaagtcagaggtggcgaaacccgacaggactataaagataccaggcgtttccccctggaagctccctcgtgcgctctcctgttccgaccctgccgcttaccggatacctgtccgcctttctcccttcgggaagcgtggcgctttctcatagctcacgctgtaggtatctcagttcggtgtaggtcgttcgctccaagctgggctgtgtgcacgaaccccccgttcagcccgaccgctgcgccttatccggtaactatcgtcttgagtccaacccggtaagacacgacttatcgccactggcagcagccactggtaacaggattagcagagcgaggtatgtaggcggtgctacagagttcttgaagtggtggcctaactacggctacactagaagaacagtatttggtatctgcgctctgctgaagccagttaccttcggaaaaagagttggtagctcttgatccggcaaacaaaccaccgctggtagcggtttttttgtttgcaagcagcagattacgcgcagaaaaaaaggatctcaagaagatcctttgatcttttctacggggtctgacgctcagtggaacgaaaactcacgttaagggattttggtcatgagattatcaaaaaggatcttcacctagatccttttaaattaaaaatgaagttttaaatcaatctaaagtatatatgagtaaacttggtctgacagttaccaatgcttaatcagtgaggcacctatctcagcgatctgtctatttcgttcatccatagttgcctgactccccgtcgtgtagataactacgatacgggagggcttaccatctggccccagtgctgcaatgataccgcgagacccacgctcaccggctccagatttatcagcaataaaccagccagccggaagggccgagcgcagaagtggtcctgcaactttatccgcctccatccagtctattaattgttgccgggaagctagagtaagtagttcgccagttaatagtttgcgcaacgttgttgccattgctacaggcatcgtggtgtcacgctcgtcgtttggtatggcttcattcagctccggttcccaacgatcaaggcgagttacatgatcccccatgttgtgcaaaaaagcggttagctccttcggtcctccgatcgttgtcagaagtaagttggccgcagtgttatcactcatggttatggcagcactgcataattctcttactgtcatgccatccgtaagatgcttttctgtgactggtgagtactcaaccaagtcattctgagaatagtgtatgcggcgaccgagttgctcttgcccggcgtcaatacgggataataccgcgccacatagcagaactttaaaagtgctcatcattggaaaacgttcttcggggcgaaaactctcaaggatcttaccgctgttgagatccagttcgatgtaacccactcgtgcacccaactgatcttcagcatcttttactttcaccagcgtttctgggtgagcaaaaacaggaaggcaaaatgccgcaaaaaagggaataagggcgacacggaaatgttgaatactcatactcttcctttttcaatattattgaagcatttatcagggttattgtctcatgagcggatacatatttgaatgtatttagaaaaataaacaaataggggttccgcgcacatttccccgaaaagtgccacctgacgtc

SEQ ID NO: 31 - DNA, 7571 bp, Artificial Sequence
  pDE1-CYB5R3-IL12B
gacggatcgggagatctcccgatcccctatggtgcactctcagtacaatctgctctgatgccgcatagttaagccagtatctgctccctgcttgtgtgttggaggtcgctgagtagtgcgcgagcaaaatttaagctacaacaaggcaaggcttgaccgacaattgcatgaagaatctgcttagggttaggcgttttgcgctgcttcgcgatgtacgggccagatatacgcgttgacattgattattgactagttattaatagtaatcaattacggggtcattagttcatagcccatatatggagttccgcgttacataacttacggtaaatggcccgcctggctgaccgcccaacgacccccgcccattgacgtcaataatgacgtatgttcccatagtaacgccaatagggactttccattgacgtcaatgggtggagtatttacggtaaactgcccacttggcagtacatcaagtgtatcatatgccaagtacgccccctattgacgtcaatgacggtaaatggcccgcctggcattatgcccagtacatgaccttatgggactttcctacttggcagtacatctacgtattagtcatcgctattaccatggtgatgcggttttggcagtacatcaatgggcgtggatagcggtttgactcacggggatttccaagtctccaccccattgacgtcaatgggagtttgttttggcaccaaaatcaacgggactttccaaaatgtcgtaacaactccgccccattgacgcaaatgggcggtaggcgtgtacggtgggaggtctatataagcagagctctctggctaactagagaacccactgcttactggcttatcgaaattaatacgactcactatagggagacccaagctggctagcgccaccatgggggcccagctcagcacgttgggccatatggtgctcttcccagtctggttcctgtacagtctgctcatgaagctgttccagcgctccacgccagccatcaccctcgagagcccggacatcaagtatcctctcagactcatcgacagagagatcattagccatgacaccagaaggttcagatttgccctgccttcaccccagcacatcctgggcctccctgtcggccagcacatctacctctcggctcgaattgatggaaacctggtcgtccggccctatacacccatctccagcgatgatgacaagggcttcgtggacctggtcatcaaggtttacttcaaggacacccatcccaagtttcccgctggagggaagatgtctcagtacctggagagcatgcagattggagacaccattgagttccggggccccagtgggctgctggtctaccagggcaaagggaagttcgccatccgacctgacaaaaagtccaaccctatcatcaggacagtgaagtctgtgggcatgatcgcgggagggacaggcatcaccccgatgctgcaggtgatccgcgccatcatgaaggaccctgatgaccacactgtgtgccacctgctctttgccaaccagaccgagaaggacatcctgctgcgacctgagctggaggaactcaggaacaaacattctgcacgcttcaagctctggtacacgctggacagagcccctgaagcctgggactacggccagggcttcgtgaatgaggagatgatccgggaccaccttccacctccagaggaggagcctctggtgctgatgtgtggacctccacctatgatccagtacgcctgccttcccaacctggaccacgtgggccaccccacggagcgctgcttcgtcttcgcctacccttacgacgtcccagactacgctggaagcggagctactaacttcagcctgctgaagcaggctggagacgtggaggagaaccctggacctaagcttggtaccatgtgtcaccagcagttggtcatctcttggttttccctggtttttctggcatctcccctcgtggccatatgggaactgaagaaagatgtttatgtcgtagaattggattggtatccggatgcccctggagaaatggtggtcctcacctgtgacacccctgaagaagatggtatcacctggaccttggaccagagcagtgaggtcttaggctctggcaaaaccctgaccatccaagtcaaagagtttggagatgctggccagtacacctgtcacaaaggaggcgaggttctatcccactctctgctgctccttcacaaaaaggaagatggaatttggtccactgatattttaaaggaccagaaagaacccaaaaataagacctttctaagatgcgaggccaagaattattctggacgtttcacctgctggtggctgacgacaatcagtactgatttgacattcagtgtcaaaagcagcagaggctcttctgacccccaaggggtgacgtgcggagctgctacactctctgcagagagagtcagaggggacaacaaggagtatgagtactcagtggagtgccaggaggacagtgcctgcccagctgctgaggagagtctgcccattgaggtcatggtggatgccgttcacaagctcaagtatgaaaactacaccagcagcttcttcatcagggacatcatcaaacctgacccacccaagaacttgcagctgaagccattaaagaattctcggcaggtggaggtcagctgggagtaccctgacacctggagtactccacattcctacttctccctgacattctgcgttcaggtccagggcaagagcaagagagaaaagaaagatagagtcttcacggacaagacctcagccacggtcatctgccgcaaaaatgccagcattagcgtgcgggcccaggaccgctactatagctcatcttggagcgaatgggcatctgtgccctgcagtggcggccgctcgagtgctggagaacagacaggagactacaaggacgacgatgacaaggcttgatctagagggcccgtttaaacccgctgatcagcctcgactgtgccttctagttgccagccatctgttgtttgcccctcccccgtgccttccttgaccctggaaggtgccactcccactgtcctttcctaataaaatgaggaaattgcatcgcattgtctgagtaggtgtcattctattctggggggtggggtggggcaggacagcaagggggaggattgggaagacaatagcaggcatgctggggatgcggtgggctctatggcttctgaggcggaaagaaccagctggggctctagggggtatccccacgcgccctgtagcggcgcattaagcgcggcgggtgtggtggttacgcgcagcgtgaccgctacacttgccagcgccctagcgcccgctcctttcgctttcttcccttcctttctcgccacgttcgccggctttccccgtcaagctctaaatcgggggctccctttagggttccgatttagtgctttacggcacctcgaccccaaaaaacttgattagggtgatggttcacgtagtgggccatcgccctgatagacggtttttcgccctttgacgttggagtccacgttctttaatagtggactcttgttccaaactggaacaacactcaaccctatctcggtctattcttttgatttataagggattttgccgatttcggcctattggttaaaaaatgagctgatttaacaaaaatttaacgcgaattaattctgtggaatgtgtgtcagttagggtgtggaaagtccccaggctccccagcaggcagaagtatgcaaagcatgcatctcaattagtcagcaaccaggtgtggaaagtccccaggctccccagcaggcagaagtatgcaaagcatgcatctcaattagtcagcaaccatagtcccgcccctaactccgcccatcccgcccctaactccgcccagttccgcccattctccgccccatggctgactaattttttttatttatgcagaggccgaggccgcctctgcctctgagctattccagaagtagtgaggaggcttttttggaggcctaggcttttgcaaaaagctcccgggagcttgtatatccattttcggatctgatcagcacgtgatgaaaaagcctgaactcaccgcgacgtctgtcgagaagtttctgatcgaaaagttcgacagcgtctccgacctgatgcagctctcggagggcgaagaatctcgtgctttcagcttcgatgtaggagggcgtggatatgtcctgcgggtaaatagctgcgccgatggtttctacaaagatcgttatgtttatcggcactttgcatcggccgcgctcccgattccggaagtgcttgacattggggaattcagcgagagcctgacctattgcatctcccgccgtgcacagggtgtcacgttgcaagacctgcctgaaaccgaactgcccgctgttctgcagccggtcgcggaggccatggatgcgatcgctgcggccgatcttagccagacgagcgggttcggcccattcggaccgcaaggaatcggtcaatacactacatggcgtgatttcatatgcgcgattgctgatccccatgtgtatcactggcaaactgtgatggacgacaccgtcagtgcgtccgtcgcgcaggctctcgatgagctgatgctttgggccgaggactgccccgaagtccggcacctcgtgcacgcggatttcggctccaacaatgtcctgacggacaatggccgcataacagcggtcattgactggagcgaggcgatgttcggggattcccaatacgaggtcgccaacatcttcttctggaggccgtggttggcttgtatggagcagcagacgcgctacttcgagcggaggcatccggagcttgcaggatcgccgcggctccgggcgtatatgctccgcattggtcttgaccaactctatcagagcttggttgacggcaatttcgatgatgcagcttgggcgcagggtcgatgcgacgcaatcgtccgatccggagccgggactgtcgggcgtacacaaatcgcccgcagaagcgcggccgtctggaccgatggctgtgtagaagtactcgccgatagtggaaaccgacgccccagcactcgtccgagggcaaaggaatagcacgtgctacgagatttcgattccaccgccgccttctatgaaaggttgggcttcggaatcgttttccgggacgccggctggatgatcctccagcgcggggatctcatgctggagttcttcgcccaccccaacttgtttattgcagcttataatggttacaaataaagcaatagcatcacaaatttcacaaataaagcatttttttcactgcattctagttgtggtttgtccaaactcatcaatgtatcttatcatgtctgtataccgtcgacctctagctagagcttggcgtaatcatggtcatagctgtttcctgtgtgaaattgttatccgctcacaattccacacaacatacgagccggaagcataaagtgtaaagcctggggtgcctaatgagtgagctaactcacattaattgcgttgcgctcactgcccgctttccagtcgggaaacctgtcgtgccagctgcattaatgaatcggccaacgcgcggggagaggcggtttgcgtattgggcgctcttccgcttcctcgctcactgactcgctgcgctcggtcgttcggctgcggcgagcggtatcagctcactcaaaggcggtaatacggttatccacagaatcaggggataacgcaggaaagaacatgtgagcaaaaggccagcaaaaggccaggaaccgtaaaaaggccgcgttgctggcgtttttccataggctccgcccccctgacgagcatcacaaaaatcgacgctcaagtcagaggtggcgaaacccgacaggactataaagataccaggcgtttccccctggaagctccctcgtgcgctctcctgttccgaccctgccgcttaccggatacctgtccgcctttctcccttcgggaagcgtggcgctttctcatagctcacgctgtaggtatctcagttcggtgtaggtcgttcgctccaagctgggctgtgtgcacgaaccccccgttcagcccgaccgctgcgccttatccggtaactatcgtcttgagtccaacccggtaagacacgacttatcgccactggcagcagccactggtaacaggattagcagagcgaggtatgtaggcggtgctacagagttcttgaagtggtggcctaactacggctacactagaagaacagtatttggtatctgcgctctgctgaagccagttaccttcggaaaaagagttggtagctcttgatccggcaaacaaaccaccgctggtagcggtttttttgtttgcaagcagcagattacgcgcagaaaaaaaggatctcaagaagatcctttgatcttttctacggggtctgacgctcagtggaacgaaaactcacgttaagggattttggtcatgagattatcaaaaaggatcttcacctagatccttttaaattaaaaatgaagttttaaatcaatctaaagtatatatgagtaaacttggtctgacagttaccaatgcttaatcagtgaggcacctatctcagcgatctgtctatttcgttcatccatagttgcctgactccccgtcgtgtagataactacgatacgggagggcttaccatctggccccagtgctgcaatgataccgcgagacccacgctcaccggctccagatttatcagcaataaaccagccagccggaagggccgagcgcagaagtggtcctgcaactttatccgcctccatccagtctattaattgttgccgggaagctagagtaagtagttcgccagttaatagtttgcgcaacgttgttgccattgctacaggcatcgtggtgtcacgctcgtcgtttggtatggcttcattcagctccggttcccaacgatcaaggcgagttacatgatcccccatgttgtgcaaaaaagcggttagctccttcggtcctccgatcgttgtcagaagtaagttggccgcagtgttatcactcatggttatggcagcactgcataattctcttactgtcatgccatccgtaagatgcttttctgtgactggtgagtactcaaccaagtcattctgagaatagtgtatgcggcgaccgagttgctcttgcccggcgtcaatacgggataataccgcgccacatagcagaactttaaaagtgctcatcattggaaaacgttcttcggggcgaaaactctcaaggatcttaccgctgttgagatccagttcgatgtaacccactcgtgcacccaactgatcttcagcatcttttactttcaccagcgtttctgggtgagcaaaaacaggaaggcaaaatgccgcaaaaaagggaataagggcgacacggaaatgttgaatactcatactcttcctttttcaatattattgaagcatttatcagggttattgtctcatgagcggatacatatttgaatgtatttagaaaaataaacaaataggggttccgcgcacatttccccgaaaagtgccacctgacgtc

SEQ ID NO: 32 - DNA, 7073 bp, Artificial Sequence
  pDE1-CYB5R3-IL15
gacggatcgggagatctcccgatcccctatggtgcactctcagtacaatctgctctgatgccgcatagttaagccagtatctgctccctgcttgtgtgttggaggtcgctgagtagtgcgcgagcaaaatttaagctacaacaaggcaaggcttgaccgacaattgcatgaagaatctgcttagggttaggcgttttgcgctgcttcgcgatgtacgggccagatatacgcgttgacattgattattgactagttattaatagtaatcaattacggggtcattagttcatagcccatatatggagttccgcgttacataacttacggtaaatggcccgcctggctgaccgcccaacgacccccgcccattgacgtcaataatgacgtatgttcccatagtaacgccaatagggactttccattgacgtcaatgggtggagtatttacggtaaactgcccacttggcagtacatcaagtgtatcatatgccaagtacgccccctattgacgtcaatgacggtaaatggcccgcctggcattatgcccagtacatgaccttatgggactttcctacttggcagtacatctacgtattagtcatcgctattaccatggtgatgcggttttggcagtacatcaatgggcgtggatagcggtttgactcacggggatttccaagtctccaccccattgacgtcaatgggagtttgttttggcaccaaaatcaacgggactttccaaaatgtcgtaacaactccgccccattgacgcaaatgggcggtaggcgtgtacggtgggaggtctatataagcagagctctctggctaactagagaacccactgcttactggcttatcgaaattaatacgactcactatagggagacccaagctggctagcgccaccatgggggcccagctcagcacgttgggccatatggtgctcttcccagtctggttcctgtacagtctgctcatgaagctgttccagcgctccacgccagccatcaccctcgagagcccggacatcaagtatcctctcagactcatcgacagagagatcattagccatgacaccagaaggttcagatttgccctgccttcaccccagcacatcctgggcctccctgtcggccagcacatctacctctcggctcgaattgatggaaacctggtcgtccggccctatacacccatctccagcgatgatgacaagggcttcgtggacctggtcatcaaggtttacttcaaggacacccatcccaagtttcccgctggagggaagatgtctcagtacctggagagcatgcagattggagacaccattgagttccggggccccagtgggctgctggtctaccagggcaaagggaagttcgccatccgacctgacaaaaagtccaaccctatcatcaggacagtgaagtctgtgggcatgatcgcgggagggacaggcatcaccccgatgctgcaggtgatccgcgccatcatgaaggaccctgatgaccacactgtgtgccacctgctctttgccaaccagaccgagaaggacatcctgctgcgacctgagctggaggaactcaggaacaaacattctgcacgcttcaagctctggtacacgctggacagagcccctgaagcctgggactacggccagggcttcgtgaatgaggagatgatccgggaccaccttccacctccagaggaggagcctctggtgctgatgtgtggacctccacctatgatccagtacgcctgccttcccaacctggaccacgtgggccaccccacggagcgctgcttcgtcttcgcctacccttacgacgtcccagactacgctggaagcggagctactaacttcagcctgctgaagcaggctggagacgtggaggagaaccctggacctaagcttggtaccatgagaatttcgaaaccacatttgagaagtatttccatccagtgctacttgtgtttacttctaaacagtcattttctaactgaagctggcattcatgtcttcattttgggctgtttcagtgcagggcttcctaaaacagaagccaactgggtgaatgtaataagtgatttgaaaaaaattgaagatcttattcaatctatgcatattgatgctactttatatacggaaagtgatgttcaccccagttgcaaagtaacagcaatgaagtgctttctcttggagttacaagttatttcacttgagtccggagatgcaagtattcatgatacagtagaaaatctgatcatcctagcaaacaacagtttgtcttctaatgggaatgtaacagaatctggatgcaaagaatgtgaggaactggaggaaaaaaatattaaagaatttttgcagagttttgtacatattgtccaaatgttcatcaacacttctggcggccgctcgagtgctggagaacagacaggagactacaaggacgacgatgacaaggcttgatctagagggcccgtttaaacccgctgatcagcctcgactgtgccttctagttgccagccatctgttgtttgcccctcccccgtgccttccttgaccctggaaggtgccactcccactgtcctttcctaataaaatgaggaaattgcatcgcattgtctgagtaggtgtcattctattctggggggtggggtggggcaggacagcaagggggaggattgggaagacaatagcaggcatgctggggatgcggtgggctctatggcttctgaggcggaaagaaccagctggggctctagggggtatccccacgcgccctgtagcggcgcattaagcgcggcgggtgtggtggttacgcgcagcgtgaccgctacacttgccagcgccctagcgcccgctcctttcgctttcttcccttcctttctcgccacgttcgccggctttccccgtcaagctctaaatcgggggctccctttagggttccgatttagtgctttacggcacctcgaccccaaaaaacttgattagggtgatggttcacgtagtgggccatcgccctgatagacggtttttcgccctttgacgttggagtccacgttctttaatagtggactcttgttccaaactggaacaacactcaaccctatctcggtctattcttttgatttataagggattttgccgatttcggcctattggttaaaaaatgagctgatttaacaaaaatttaacgcgaattaattctgtggaatgtgtgtcagttagggtgtggaaagtccccaggctccccagcaggcagaagtatgcaaagcatgcatctcaattagtcagcaaccaggtgtggaaagtccccaggctccccagcaggcagaagtatgcaaagcatgcatctcaattagtcagcaaccatagtcccgcccctaactccgcccatcccgcccctaactccgcccagttccgcccattctccgccccatggctgactaattttttttatttatgcagaggccgaggccgcctctgcctctgagctattccagaagtagtgaggaggcttttttggaggcctaggcttttgcaaaaagctcccgggagcttgtatatccattttcggatctgatcagcacgtgatgaaaaagcctgaactcaccgcgacgtctgtcgagaagtttctgatcgaaaagttcgacagcgtctccgacctgatgcagctctcggagggcgaagaatctcgtgctttcagcttcgatgtaggagggcgtggatatgtcctgcgggtaaatagctgcgccgatggtttctacaaagatcgttatgtttatcggcactttgcatcggccgcgctcccgattccggaagtgcttgacattggggaattcagcgagagcctgacctattgcatctcccgccgtgcacagggtgtcacgttgcaagacctgcctgaaaccgaactgcccgctgttctgcagccggtcgcggaggccatggatgcgatcgctgcggccgatcttagccagacgagcgggttcggcccattcggaccgcaaggaatcggtcaatacactacatggcgtgatttcatatgcgcgattgctgatccccatgtgtatcactggcaaactgtgatggacgacaccgtcagtgcgtccgtcgcgcaggctctcgatgagctgatgctttgggccgaggactgccccgaagtccggcacctcgtgcacgcggatttcggctccaacaatgtcctgacggacaatggccgcataacagcggtcattgactggagcgaggcgatgttcggggattcccaatacgaggtcgccaacatcttcttctggaggccgtggttggcttgtatggagcagcagacgcgctacttcgagcggaggcatccggagcttgcaggatcgccgcggctccgggcgtatatgctccgcattggtcttgaccaactctatcagagcttggttgacggcaatttcgatgatgcagcttgggcgcagggtcgatgcgacgcaatcgtccgatccggagccgggactgtcgggcgtacacaaatcgcccgcagaagcgcggccgtctggaccgatggctgtgtagaagtactcgccgatagtggaaaccgacgccccagcactcgtccgagggcaaaggaatagcacgtgctacgagatttcgattccaccgccgccttctatgaaaggttgggcttcggaatcgttttccgggacgccggctggatgatcctccagcgcggggatctcatgctggagttcttcgcccaccccaacttgtttattgcagcttataatggttacaaataaagcaatagcatcacaaatttcacaaataaagcatttttttcactgcattctagttgtggtttgtccaaactcatcaatgtatcttatcatgtctgtataccgtcgacctctagctagagcttggcgtaatcatggtcatagctgtttcctgtgtgaaattgttatccgctcacaattccacacaacatacgagccggaagcataaagtgtaaagcctggggtgcctaatgagtgagctaactcacattaattgcgttgcgctcactgcccgctttccagtcgggaaacctgtcgtgccagctgcattaatgaatcggccaacgcgcggggagaggcggtttgcgtattgggcgctcttccgcttcctcgctcactgactcgctgcgctcggtcgttcggctgcggcgagcggtatcagctcactcaaaggcggtaatacggttatccacagaatcaggggataacgcaggaaagaacatgtgagcaaaaggccagcaaaaggccaggaaccgtaaaaaggccgcgttgctggcgtttttccataggctccgcccccctgacgagcatcacaaaaatcgacgctcaagtcagaggtggcgaaacccgacaggactataaagataccaggcgtttccccctggaagctccctcgtgcgctctcctgttccgaccctgccgcttaccggatacctgtccgcctttctcccttcgggaagcgtggcgctttctcatagctcacgctgtaggtatctcagttcggtgtaggtcgttcgctccaagctgggctgtgtgcacgaaccccccgttcagcccgaccgctgcgccttatccggtaactatcgtcttgagtccaacccggtaagacacgacttatcgccactggcagcagccactggtaacaggattagcagagcgaggtatgtaggcggtgctacagagttcttgaagtggtggcctaactacggctacactagaagaacagtatttggtatctgcgctctgctgaagccagttaccttcggaaaaagagttggtagctcttgatccggcaaacaaaccaccgctggtagcggtttttttgtttgcaagcagcagattacgcgcagaaaaaaaggatctcaagaagatcctttgatcttttctacggggtctgacgctcagtggaacgaaaactcacgttaagggattttggtcatgagattatcaaaaaggatcttcacctagatccttttaaattaaaaatgaagttttaaatcaatctaaagtatatatgagtaaacttggtctgacagttaccaatgcttaatcagtgaggcacctatctcagcgatctgtctatttcgttcatccatagttgcctgactccccgtcgtgtagataactacgatacgggagggcttaccatctggccccagtgctgcaatgataccgcgagacccacgctcaccggctccagatttatcagcaataaaccagccagccggaagggccgagcgcagaagtggtcctgcaactttatccgcctccatccagtctattaattgttgccgggaagctagagtaagtagttcgccagttaatagtttgcgcaacgttgttgccattgctacaggcatcgtggtgtcacgctcgtcgtttggtatggcttcattcagctccggttcccaacgatcaaggcgagttacatgatcccccatgttgtgcaaaaaagcggttagctccttcggtcctccgatcgttgtcagaagtaagttggccgcagtgttatcactcatggttatggcagcactgcataattctcttactgtcatgccatccgtaagatgcttttctgtgactggtgagtactcaaccaagtcattctgagaatagtgtatgcggcgaccgagttgctcttgcccggcgtcaatacgggataataccgcgccacatagcagaactttaaaagtgctcatcattggaaaacgttcttcggggcgaaaactctcaaggatcttaccgctgttgagatccagttcgatgtaacccactcgtgcacccaactgatcttcagcatcttttactttcaccagcgtttctgggtgagcaaaaacaggaaggcaaaatgccgcaaaaaagggaataagggcgacacggaaatgttgaatactcatactcttcctttttcaatattattgaagcatttatcagggttattgtctcatgagcggatacatatttgaatgtatttagaaaaataaacaaataggggttccgcgcacatttccccgaaaagtgccacctgacgtc

SEQ ID NO: 33 - DNA, 7073 bp, Artificial Sequence
  pDE1-CYB5R3-IL21
gacggatcgggagatctcccgatcccctatggtgcactctcagtacaatctgctctgatgccgcatagttaagccagtatctgctccctgcttgtgtgttggaggtcgctgagtagtgcgcgagcaaaatttaagctacaacaaggcaaggcttgaccgacaattgcatgaagaatctgcttagggttaggcgttttgcgctgcttcgcgatgtacgggccagatatacgcgttgacattgattattgactagttattaatagtaatcaattacggggtcattagttcatagcccatatatggagttccgcgttacataacttacggtaaatggcccgcctggctgaccgcccaacgacccccgcccattgacgtcaataatgacgtatgttcccatagtaacgccaatagggactttccattgacgtcaatgggtggagtatttacggtaaactgcccacttggcagtacatcaagtgtatcatatgccaagtacgccccctattgacgtcaatgacggtaaatggcccgcctggcattatgcccagtacatgaccttatgggactttcctacttggcagtacatctacgtattagtcatcgctattaccatggtgatgcggttttggcagtacatcaatgggcgtggatagcggtttgactcacggggatttccaagtctccaccccattgacgtcaatgggagtttgttttggcaccaaaatcaacgggactttccaaaatgtcgtaacaactccgccccattgacgcaaatgggcggtaggcgtgtacggtgggaggtctatataagcagagctctctggctaactagagaacccactgcttactggcttatcgaaattaatacgactcactatagggagacccaagctggctagcgccaccatgggggcccagctcagcacgttgggccatatggtgctcttcccagtctggttcctgtacagtctgctcatgaagctgttccagcgctccacgccagccatcaccctcgagagcccggacatcaagtatcctctcagactcatcgacagagagatcattagccatgacaccagaaggttcagatttgccctgccttcaccccagcacatcctgggcctccctgtcggccagcacatctacctctcggctcgaattgatggaaacctggtcgtccggccctatacacccatctccagcgatgatgacaagggcttcgtggacctggtcatcaaggtttacttcaaggacacccatcccaagtttcccgctggagggaagatgtctcagtacctggagagcatgcagattggagacaccattgagttccggggccccagtgggctgctggtctaccagggcaaagggaagttcgccatccgacctgacaaaaagtccaaccctatcatcaggacagtgaagtctgtgggcatgatcgcgggagggacaggcatcaccccgatgctgcaggtgatccgcgccatcatgaaggaccctgatgaccacactgtgtgccacctgctctttgccaaccagaccgagaaggacatcctgctgcgacctgagctggaggaactcaggaacaaacattctgcacgcttcaagctctggtacacgctggacagagcccctgaagcctgggactacggccagggcttcgtgaatgaggagatgatccgggaccaccttccacctccagaggaggagcctctggtgctgatgtgtggacctccacctatgatccagtacgcctgccttcccaacctggaccacgtgggccaccccacggagcgctgcttcgtcttcgcctacccttacgacgtcccagactacgctggaagcggagctactaacttcagcctgctgaagcaggctggagacgtggaggagaaccctggacctaagcttggtaccatgagatccagtcctggcaacatggagaggattgtcatctgtctgatggtcatcttcttggggacactggtccacaaatcaagctcccaaggtcaagatcgccacatgattagaatgcgtcaacttatagatattgttgatcagctgaaaaattatgtgaatgacttggtccctgaatttctgccagctccagaagatgtagagacaaactgtgagtggtcagctttttcctgctttcagaaggcccaactaaagtcagcaaatacaggaaacaatgaaaggataatcaatgtatcaattaaaaagctgaagaggaaaccaccttccacaaatgcagggagaagacagaaacacagactaacatgcccttcatgtgattcttatgagaaaaaaccacccaaagaattcctagaaagattcaaatcacttctccaaaagatgattcatcagcatctgtcctctagaacacacggaagtgaagattccggcggccgctcgagtgctggagaacagacaggagactacaaggacgacgatgacaaggcttgatctagagggcccgtttaaacccgctgatcagcctcgactgtgccttctagttgccagccatctgttgtttgcccctcccccgtgccttccttgaccctggaaggtgccactcccactgtcctttcctaataaaatgaggaaattgcatcgcattgtctgagtaggtgtcattctattctggggggtggggtggggcaggacagcaagggggaggattgggaagacaatagcaggcatgctggggatgcggtgggctctatggcttctgaggcggaaagaaccagctggggctctagggggtatccccacgcgccctgtagcggcgcattaagcgcggcgggtgtggtggttacgcgcagcgtgaccgctacacttgccagcgccctagcgcccgctcctttcgctttcttcccttcctttctcgccacgttcgccggctttccccgtcaagctctaaatcgggggctccctttagggttccgatttagtgctttacggcacctcgaccccaaaaaacttgattagggtgatggttcacgtagtgggccatcgccctgatagacggtttttcgccctttgacgttggagtccacgttctttaatagtggactcttgttccaaactggaacaacactcaaccctatctcggtctattcttttgatttataagggattttgccgatttcggcctattggttaaaaaatgagctgatttaacaaaaatttaacgcgaattaattctgtggaatgtgtgtcagttagggtgtggaaagtccccaggctccccagcaggcagaagtatgcaaagcatgcatctcaattagtcagcaaccaggtgtggaaagtccccaggctccccagcaggcagaagtatgcaaagcatgcatctcaattagtcagcaaccatagtcccgcccctaactccgcccatcccgcccctaactccgcccagttccgcccattctccgccccatggctgactaattttttttatttatgcagaggccgaggccgcctctgcctctgagctattccagaagtagtgaggaggcttttttggaggcctaggcttttgcaaaaagctcccgggagcttgtatatccattttcggatctgatcagcacgtgatgaaaaagcctgaactcaccgcgacgtctgtcgagaagtttctgatcgaaaagttcgacagcgtctccgacctgatgcagctctcggagggcgaagaatctcgtgctttcagcttcgatgtaggagggcgtggatatgtcctgcgggtaaatagctgcgccgatggtttctacaaagatcgttatgtttatcggcactttgcatcggccgcgctcccgattccggaagtgcttgacattggggaattcagcgagagcctgacctattgcatctcccgccgtgcacagggtgtcacgttgcaagacctgcctgaaaccgaactgcccgctgttctgcagccggtcgcggaggccatggatgcgatcgctgcggccgatcttagccagacgagcgggttcggcccattcggaccgcaaggaatcggtcaatacactacatggcgtgatttcatatgcgcgattgctgatccccatgtgtatcactggcaaactgtgatggacgacaccgtcagtgcgtccgtcgcgcaggctctcgatgagctgatgctttgggccgaggactgccccgaagtccggcacctcgtgcacgcggatttcggctccaacaatgtcctgacggacaatggccgcataacagcggtcattgactggagcgaggcgatgttcggggattcccaatacgaggtcgccaacatcttcttctggaggccgtggttggcttgtatggagcagcagacgcgctacttcgagcggaggcatccggagcttgcaggatcgccgcggctccgggcgtatatgctccgcattggtcttgaccaactctatcagagcttggttgacggcaatttcgatgatgcagcttgggcgcagggtcgatgcgacgcaatcgtccgatccggagccgggactgtcgggcgtacacaaatcgcccgcagaagcgcggccgtctggaccgatggctgtgtagaagtactcgccgatagtggaaaccgacgccccagcactcgtccgagggcaaaggaatagcacgtgctacgagatttcgattccaccgccgccttctatgaaaggttgggcttcggaatcgttttccgggacgccggctggatgatcctccagcgcggggatctcatgctggagttcttcgcccaccccaacttgtttattgcagcttataatggttacaaataaagcaatagcatcacaaatttcacaaataaagcatttttttcactgcattctagttgtggtttgtccaaactcatcaatgtatcttatcatgtctgtataccgtcgacctctagctagagcttggcgtaatcatggtcatagctgtttcctgtgtgaaattgttatccgctcacaattccacacaacatacgagccggaagcataaagtgtaaagcctggggtgcctaatgagtgagctaactcacattaattgcgttgcgctcactgcccgctttccagtcgggaaacctgtcgtgccagctgcattaatgaatcggccaacgcgcggggagaggcggtttgcgtattgggcgctcttccgcttcctcgctcactgactcgctgcgctcggtcgttcggctgcggcgagcggtatcagctcactcaaaggcggtaatacggttatccacagaatcaggggataacgcaggaaagaacatgtgagcaaaaggccagcaaaaggccaggaaccgtaaaaaggccgcgttgctggcgtttttccataggctccgcccccctgacgagcatcacaaaaatcgacgctcaagtcagaggtggcgaaacccgacaggactataaagataccaggcgtttccccctggaagctccctcgtgcgctctcctgttccgaccctgccgcttaccggatacctgtccgcctttctcccttcgggaagcgtggcgctttctcatagctcacgctgtaggtatctcagttcggtgtaggtcgttcgctccaagctgggctgtgtgcacgaaccccccgttcagcccgaccgctgcgccttatccggtaactatcgtcttgagtccaacccggtaagacacgacttatcgccactggcagcagccactggtaacaggattagcagagcgaggtatgtaggcggtgctacagagttcttgaagtggtggcctaactacggctacactagaagaacagtatttggtatctgcgctctgctgaagccagttaccttcggaaaaagagttggtagctcttgatccggcaaacaaaccaccgctggtagcggtttttttgtttgcaagcagcagattacgcgcagaaaaaaaggatctcaagaagatcctttgatcttttctacggggtctgacgctcagtggaacgaaaactcacgttaagggattttggtcatgagattatcaaaaaggatcttcacctagatccttttaaattaaaaatgaagttttaaatcaatctaaagtatatatgagtaaacttggtctgacagttaccaatgcttaatcagtgaggcacctatctcagcgatctgtctatttcgttcatccatagttgcctgactccccgtcgtgtagataactacgatacgggagggcttaccatctggccccagtgctgcaatgataccgcgagacccacgctcaccggctccagatttatcagcaataaaccagccagccggaagggccgagcgcagaagtggtcctgcaactttatccgcctccatccagtctattaattgttgccgggaagctagagtaagtagttcgccagttaatagtttgcgcaacgttgttgccattgctacaggcatcgtggtgtcacgctcgtcgtttggtatggcttcattcagctccggttcccaacgatcaaggcgagttacatgatcccccatgttgtgcaaaaaagcggttagctccttcggtcctccgatcgttgtcagaagtaagttggccgcagtgttatcactcatggttatggcagcactgcataattctcttactgtcatgccatccgtaagatgcttttctgtgactggtgagtactcaaccaagtcattctgagaatagtgtatgcggcgaccgagttgctcttgcccggcgtcaatacgggataataccgcgccacatagcagaactttaaaagtgctcatcattggaaaacgttcttcggggcgaaaactctcaaggatcttaccgctgttgagatccagttcgatgtaacccactcgtgcacccaactgatcttcagcatcttttactttcaccagcgtttctgggtgagcaaaaacaggaaggcaaaatgccgcaaaaaagggaataagggcgacacggaaatgttgaatactcatactcttcctttttcaatattattgaagcatttatcagggttattgtctcatgagcggatacatatttgaatgtatttagaaaaataaacaaataggggttccgcgcacatttccccgaaaagtgccacctgacgtc

SEQ ID NO: 34 - DNA, 7241 bp, Artificial Sequence
  pDE1-CYB5R3-IL37
gacggatcgggagatctcccgatcccctatggtgcactctcagtacaatctgctctgatgccgcatagttaagccagtatctgctccctgcttgtgtgttggaggtcgctgagtagtgcgcgagcaaaatttaagctacaacaaggcaaggcttgaccgacaattgcatgaagaatctgcttagggttaggcgttttgcgctgcttcgcgatgtacgggccagatatacgcgttgacattgattattgactagttattaatagtaatcaattacggggtcattagttcatagcccatatatggagttccgcgttacataacttacggtaaatggcccgcctggctgaccgcccaacgacccccgcccattgacgtcaataatgacgtatgttcccatagtaacgccaatagggactttccattgacgtcaatgggtggagtatttacggtaaactgcccacttggcagtacatcaagtgtatcatatgccaagtacgccccctattgacgtcaatgacggtaaatggcccgcctggcattatgcccagtacatgaccttatgggactttcctacttggcagtacatctacgtattagtcatcgctattaccatggtgatgcggttttggcagtacatcaatgggcgtggatagcggtttgactcacggggatttccaagtctccaccccattgacgtcaatgggagtttgttttggcaccaaaatcaacgggactttccaaaatgtcgtaacaactccgccccattgacgcaaatgggcggtaggcgtgtacggtgggaggtctatataagcagagctctctggctaactagagaacccactgcttactggcttatcgaaattaatacgactcactatagggagacccaagctggctagcgccaccatgggggcccagctcagcacgttgggccatatggtgctcttcccagtctggttcctgtacagtctgctcatgaagctgttccagcgctccacgccagccatcaccctcgagagcccggacatcaagtatcctctcagactcatcgacagagagatcattagccatgacaccagaaggttcagatttgccctgccttcaccccagcacatcctgggcctccctgtcggccagcacatctacctctcggctcgaattgatggaaacctggtcgtccggccctatacacccatctccagcgatgatgacaagggcttcgtggacctggtcatcaaggtttacttcaaggacacccatcccaagtttcccgctggagggaagatgtctcagtacctggagagcatgcagattggagacaccattgagttccggggccccagtgggctgctggtctaccagggcaaagggaagttcgccatccgacctgacaaaaagtccaaccctatcatcaggacagtgaagtctgtgggcatgatcgcgggagggacaggcatcaccccgatgctgcaggtgatccgcgccatcatgaaggaccctgatgaccacactgtgtgccacctgctctttgccaaccagaccgagaaggacatcctgctgcgacctgagctggaggaactcaggaacaaacattctgcacgcttcaagctctggtacacgctggacagagcccctgaagcctgggactacggccagggcttcgtgaatgaggagatgatccgggaccaccttccacctccagaggaggagcctctggtgctgatgtgtggacctccacctatgatccagtacgcctgccttcccaacctggaccacgtgggccaccccacggagcgctgcttcgtcttcgcctacccttacgacgtcccagactacgctggaagcggagctactaacttcagcctgctgaagcaggctggagacgtggaggagaaccctggacctaagcttggtaccatgtcctttgtgggggagaactcaggagtgaaaatgggctctgaggactgggaaaaagatgaaccccagtgctgcttagaagacccggctggaagccccctggaaccaggcccaagcctccccaccatgaattttgttcacacaagtccaaaggtgaagaacttaaacccgaagaaattcagcattcatgaccaggatcacaaagtactggtcctggactctgggaatctcatagcagttccagataaaaactacatacgcccagagatcttctttgcattagcctcatccttgagctcagcctctgcggagaaaggaagtccgattctcctgggggtctctaaaggggagttttgtctctactgtgacaaggataaaggacaaagtcatccatcccttcagctgaagaaggagaaactgatgaagctggctgcccaaaaggaatcagcacgccggcccttcatcttttatagggctcaggtgggctcctggaacatgctggagtcggcggctcaccccggatggttcatctgcacctcctgcaattgtaatgagcctgttggggtgacagataaatttgagaacaggaaacacattgaattttcatttcaaccagtttgcaaagctgaaatgagccccagtgaggtcagcgatggcggccgctcgagtgctggagaacagacaggagactacaaggacgacgatgacaaggcttgatctagagggcccgtttaaacccgctgatcagcctcgactgtgccttctagttgccagccatctgttgtttgcccctcccccgtgccttccttgaccctggaaggtgccactcccactgtcctttcctaataaaatgaggaaattgcatcgcattgtctgagtaggtgtcattctattctggggggtggggtggggcaggacagcaagggggaggattgggaagacaatagcaggcatgctggggatgcggtgggctctatggcttctgaggcggaaagaaccagctggggctctagggggtatccccacgcgccctgtagcggcgcattaagcgcggcgggtgtggtggttacgcgcagcgtgaccgctacacttgccagcgccctagcgcccgctcctttcgctttcttcccttcctttctcgccacgttcgccggctttccccgtcaagctctaaatcgggggctccctttagggttccgatttagtgctttacggcacctcgaccccaaaaaacttgattagggtgatggttcacgtagtgggccatcgccctgatagacggtttttcgccctttgacgttggagtccacgttctttaatagtggactcttgttccaaactggaacaacactcaaccctatctcggtctattcttttgatttataagggattttgccgatttcggcctattggttaaaaaatgagctgatttaacaaaaatttaacgcgaattaattctgtggaatgtgtgtcagttagggtgtggaaagtccccaggctccccagcaggcagaagtatgcaaagcatgcatctcaattagtcagcaaccaggtgtggaaagtccccaggctccccagcaggcagaagtatgcaaagcatgcatctcaattagtcagcaaccatagtcccgcccctaactccgcccatcccgcccctaactccgcccagttccgcccattctccgccccatggctgactaattttttttatttatgcagaggccgaggccgcctctgcctctgagctattccagaagtagtgaggaggcttttttggaggcctaggcttttgcaaaaagctcccgggagcttgtatatccattttcggatctgatcagcacgtgatgaaaaagcctgaactcaccgcgacgtctgtcgagaagtttctgatcgaaaagttcgacagcgtctccgacctgatgcagctctcggagggcgaagaatctcgtgctttcagcttcgatgtaggagggcgtggatatgtcctgcgggtaaatagctgcgccgatggtttctacaaagatcgttatgtttatcggcactttgcatcggccgcgctcccgattccggaagtgcttgacattggggaattcagcgagagcctgacctattgcatctcccgccgtgcacagggtgtcacgttgcaagacctgcctgaaaccgaactgcccgctgttctgcagccggtcgcggaggccatggatgcgatcgctgcggccgatcttagccagacgagcgggttcggcccattcggaccgcaaggaatcggtcaatacactacatggcgtgatttcatatgcgcgattgctgatccccatgtgtatcactggcaaactgtgatggacgacaccgtcagtgcgtccgtcgcgcaggctctcgatgagctgatgctttgggccgaggactgccccgaagtccggcacctcgtgcacgcggatttcggctccaacaatgtcctgacggacaatggccgcataacagcggtcattgactggagcgaggcgatgttcggggattcccaatacgaggtcgccaacatcttcttctggaggccgtggttggcttgtatggagcagcagacgcgctacttcgagcggaggcatccggagcttgcaggatcgccgcggctccgggcgtatatgctccgcattggtcttgaccaactctatcagagcttggttgacggcaatttcgatgatgcagcttgggcgcagggtcgatgcgacgcaatcgtccgatccggagccgggactgtcgggcgtacacaaatcgcccgcagaagcgcggccgtctggaccgatggctgtgtagaagtactcgccgatagtggaaaccgacgccccagcactcgtccgagggcaaaggaatagcacgtgctacgagatttcgattccaccgccgccttctatgaaaggttgggcttcggaatcgttttccgggacgccggctggatgatcctccagcgcggggatctcatgctggagttcttcgcccaccccaacttgtttattgcagcttataatggttacaaataaagcaatagcatcacaaatttcacaaataaagcatttttttcactgcattctagttgtggtttgtccaaactcatcaatgtatcttatcatgtctgtataccgtcgacctctagctagagcttggcgtaatcatggtcatagctgtttcctgtgtgaaattgttatccgctcacaattccacacaacatacgagccggaagcataaagtgtaaagcctggggtgcctaatgagtgagctaactcacattaattgcgttgcgctcactgcccgctttccagtcgggaaacctgtcgtgccagctgcattaatgaatcggccaacgcgcggggagaggcggtttgcgtattgggcgctcttccgcttcctcgctcactgactcgctgcgctcggtcgttcggctgcggcgagcggtatcagctcactcaaaggcggtaatacggttatccacagaatcaggggataacgcaggaaagaacatgtgagcaaaaggccagcaaaaggccaggaaccgtaaaaaggccgcgttgctggcgtttttccataggctccgcccccctgacgagcatcacaaaaatcgacgctcaagtcagaggtggcgaaacccgacaggactataaagataccaggcgtttccccctggaagctccctcgtgcgctctcctgttccgaccctgccgcttaccggatacctgtccgcctttctcccttcgggaagcgtggcgctttctcatagctcacgctgtaggtatctcagttcggtgtaggtcgttcgctccaagctgggctgtgtgcacgaaccccccgttcagcccgaccgctgcgccttatccggtaactatcgtcttgagtccaacccggtaagacacgacttatcgccactggcagcagccactggtaacaggattagcagagcgaggtatgtaggcggtgctacagagttcttgaagtggtggcctaactacggctacactagaagaacagtatttggtatctgcgctctgctgaagccagttaccttcggaaaaagagttggtagctcttgatccggcaaacaaaccaccgctggtagcggtttttttgtttgcaagcagcagattacgcgcagaaaaaaaggatctcaagaagatcctttgatcttttctacggggtctgacgctcagtggaacgaaaactcacgttaagggattttggtcatgagattatcaaaaaggatcttcacctagatccttttaaattaaaaatgaagttttaaatcaatctaaagtatatatgagtaaacttggtctgacagttaccaatgcttaatcagtgaggcacctatctcagcgatctgtctatttcgttcatccatagttgcctgactccccgtcgtgtagataactacgatacgggagggcttaccatctggccccagtgctgcaatgataccgcgagacccacgctcaccggctccagatttatcagcaataaaccagccagccggaagggccgagcgcagaagtggtcctgcaactttatccgcctccatccagtctattaattgttgccgggaagctagagtaagtagttcgccagttaatagtttgcgcaacgttgttgccattgctacaggcatcgtggtgtcacgctcgtcgtttggtatggcttcattcagctccggttcccaacgatcaaggcgagttacatgatcccccatgttgtgcaaaaaagcggttagctccttcggtcctccgatcgttgtcagaagtaagttggccgcagtgttatcactcatggttatggcagcactgcataattctcttactgtcatgccatccgtaagatgcttttctgtgactggtgagtactcaaccaagtcattctgagaatagtgtatgcggcgaccgagttgctcttgcccggcgtcaatacgggataataccgcgccacatagcagaactttaaaagtgctcatcattggaaaacgttcttcggggcgaaaactctcaaggatcttaccgctgttgagatccagttcgatgtaacccactcgtgcacccaactgatcttcagcatcttttactttcaccagcgtttctgggtgagcaaaaacaggaaggcaaaatgccgcaaaaaagggaataagggcgacacggaaatgttgaatactcatactcttcctttttcaatattattgaagcatttatcagggttattgtctcatgagcggatacatatttgaatgtatttagaaaaataaacaaataggggttccgcgcacatttccccgaaaagtgccacctgacgtc

SEQ ID NO: 35 - DNA, 7019 bp, Artificial Sequence
  pDE1-CYB5R3-GMCSF
gacggatcgggagatctcccgatcccctatggtgcactctcagtacaatctgctctgatgccgcatagttaagccagtatctgctccctgcttgtgtgttggaggtcgctgagtagtgcgcgagcaaaatttaagctacaacaaggcaaggcttgaccgacaattgcatgaagaatctgcttagggttaggcgttttgcgctgcttcgcgatgtacgggccagatatacgcgttgacattgattattgactagttattaatagtaatcaattacggggtcattagttcatagcccatatatggagttccgcgttacataacttacggtaaatggcccgcctggctgaccgcccaacgacccccgcccattgacgtcaataatgacgtatgttcccatagtaacgccaatagggactttccattgacgtcaatgggtggagtatttacggtaaactgcccacttggcagtacatcaagtgtatcatatgccaagtacgccccctattgacgtcaatgacggtaaatggcccgcctggcattatgcccagtacatgaccttatgggactttcctacttggcagtacatctacgtattagtcatcgctattaccatggtgatgcggttttggcagtacatcaatgggcgtggatagcggtttgactcacggggatttccaagtctccaccccattgacgtcaatgggagtttgttttggcaccaaaatcaacgggactttccaaaatgtcgtaacaactccgccccattgacgcaaatgggcggtaggcgtgtacggtgggaggtctatataagcagagctctctggctaactagagaacccactgcttactggcttatcgaaattaatacgactcactatagggagacccaagctggctagcgccaccatgggggcccagctcagcacgttgggccatatggtgctcttcccagtctggttcctgtacagtctgctcatgaagctgttccagcgctccacgccagccatcaccctcgagagcccggacatcaagtatcctctcagactcatcgacagagagatcattagccatgacaccagaaggttcagatttgccctgccttcaccccagcacatcctgggcctccctgtcggccagcacatctacctctcggctcgaattgatggaaacctggtcgtccggccctatacacccatctccagcgatgatgacaagggcttcgtggacctggtcatcaaggtttacttcaaggacacccatcccaagtttcccgctggagggaagatgtctcagtacctggagagcatgcagattggagacaccattgagttccggggccccagtgggctgctggtctaccagggcaaagggaagttcgccatccgacctgacaaaaagtccaaccctatcatcaggacagtgaagtctgtgggcatgatcgcgggagggacaggcatcaccccgatgctgcaggtgatccgcgccatcatgaaggaccctgatgaccacactgtgtgccacctgctctttgccaaccagaccgagaaggacatcctgctgcgacctgagctggaggaactcaggaacaaacattctgcacgcttcaagctctggtacacgctggacagagcccctgaagcctgggactacggccagggcttcgtgaatgaggagatgatccgggaccaccttccacctccagaggaggagcctctggtgctgatgtgtggacctccacctatgatccagtacgcctgccttcccaacctggaccacgtgggccaccccacggagcgctgcttcgtcttcgcctacccttacgacgtcccagactacgctggaagcggagctactaacttcagcctgctgaagcaggctggagacgtggaggagaaccctggacctaagcttggtaccatgtggctgcagagcctgctgctccttggaactgtggcttgttctatctctgcacctgctcgcagtccatctcctagcactcagccatgggagcatgtgaatgccatccaggaggcccggcgtctcctgaacctgagtagagacactgctgctgagatgaatgaaacagtagaagtcatctcagaaatgtttgatcttcaggagccgacatgcctacagacaagactggagctgtacaagcagggactgagaggatctttgacaaagctcaagggccccttgaccatgatggccagccactacaagcagcactgccctccaaccccggaaacttcctgtgcaacccagattatcacctttgaaagtttcaaagagaacctgaaggactttctgcttgtcatcccctttgactgctgggagccagtccaggagggcggccgctcgagtgctggagaacagacaggagactacaaggacgacgatgacaaggcttgatctagagggcccgtttaaacccgctgatcagcctcgactgtgccttctagttgccagccatctgttgtttgcccctcccccgtgccttccttgaccctggaaggtgccactcccactgtcctttcctaataaaatgaggaaattgcatcgcattgtctgagtaggtgtcattctattctggggggtggggtggggcaggacagcaagggggaggattgggaagacaatagcaggcatgctggggatgcggtgggctctatggcttctgaggcggaaagaaccagctggggctctagggggtatccccacgcgccctgtagcggcgcattaagcgcggcgggtgtggtggttacgcgcagcgtgaccgctacacttgccagcgccctagcgcccgctcctttcgctttcttcccttcctttctcgccacgttcgccggctttccccgtcaagctctaaatcgggggctccctttagggttccgatttagtgctttacggcacctcgaccccaaaaaacttgattagggtgatggttcacgtagtgggccatcgccctgatagacggtttttcgccctttgacgttggagtccacgttctttaatagtggactcttgttccaaactggaacaacactcaaccctatctcggtctattcttttgatttataagggattttgccgatttcggcctattggttaaaaaatgagctgatttaacaaaaatttaacgcgaattaattctgtggaatgtgtgtcagttagggtgtggaaagtccccaggctccccagcaggcagaagtatgcaaagcatgcatctcaattagtcagcaaccaggtgtggaaagtccccaggctccccagcaggcagaagtatgcaaagcatgcatctcaattagtcagcaaccatagtcccgcccctaactccgcccatcccgcccctaactccgcccagttccgcccattctccgccccatggctgactaattttttttatttatgcagaggccgaggccgcctctgcctctgagctattccagaagtagtgaggaggcttttttggaggcctaggcttttgcaaaaagctcccgggagcttgtatatccattttcggatctgatcagcacgtgatgaaaaagcctgaactcaccgcgacgtctgtcgagaagtttctgatcgaaaagttcgacagcgtctccgacctgatgcagctctcggagggcgaagaatctcgtgctttcagcttcgatgtaggagggcgtggatatgtcctgcgggtaaatagctgcgccgatggtttctacaaagatcgttatgtttatcggcactttgcatcggccgcgctcccgattccggaagtgcttgacattggggaattcagcgagagcctgacctattgcatctcccgccgtgcacagggtgtcacgttgcaagacctgcctgaaaccgaactgcccgctgttctgcagccggtcgcggaggccatggatgcgatcgctgcggccgatcttagccagacgagcgggttcggcccattcggaccgcaaggaatcggtcaatacactacatggcgtgatttcatatgcgcgattgctgatccccatgtgtatcactggcaaactgtgatggacgacaccgtcagtgcgtccgtcgcgcaggctctcgatgagctgatgctttgggccgaggactgccccgaagtccggcacctcgtgcacgcggatttcggctccaacaatgtcctgacggacaatggccgcataacagcggtcattgactggagcgaggcgatgttcggggattcccaatacgaggtcgccaacatcttcttctggaggccgtggttggcttgtatggagcagcagacgcgctacttcgagcggaggcatccggagcttgcaggatcgccgcggctccgggcgtatatgctccgcattggtcttgaccaactctatcagagcttggttgacggcaatttcgatgatgcagcttgggcgcagggtcgatgcgacgcaatcgtccgatccggagccgggactgtcgggcgtacacaaatcgcccgcagaagcgcggccgtctggaccgatggctgtgtagaagtactcgccgatagtggaaaccgacgccccagcactcgtccgagggcaaaggaatagcacgtgctacgagatttcgattccaccgccgccttctatgaaaggttgggcttcggaatcgttttccgggacgccggctggatgatcctccagcgcggggatctcatgctggagttcttcgcccaccccaacttgtttattgcagcttataatggttacaaataaagcaatagcatcacaaatttcacaaataaagcatttttttcactgcattctagttgtggtttgtccaaactcatcaatgtatcttatcatgtctgtataccgtcgacctctagctagagcttggcgtaatcatggtcatagctgtttcctgtgtgaaattgttatccgctcacaattccacacaacatacgagccggaagcataaagtgtaaagcctggggtgcctaatgagtgagctaactcacattaattgcgttgcgctcactgcccgctttccagtcgggaaacctgtcgtgccagctgcattaatgaatcggccaacgcgcggggagaggcggtttgcgtattgggcgctcttccgcttcctcgctcactgactcgctgcgctcggtcgttcggctgcggcgagcggtatcagctcactcaaaggcggtaatacggttatccacagaatcaggggataacgcaggaaagaacatgtgagcaaaaggccagcaaaaggccaggaaccgtaaaaaggccgcgttgctggcgtttttccataggctccgcccccctgacgagcatcacaaaaatcgacgctcaagtcagaggtggcgaaacccgacaggactataaagataccaggcgtttccccctggaagctccctcgtgcgctctcctgttccgaccctgccgcttaccggatacctgtccgcctttctcccttcgggaagcgtggcgctttctcatagctcacgctgtaggtatctcagttcggtgtaggtcgttcgctccaagctgggctgtgtgcacgaaccccccgttcagcccgaccgctgcgccttatccggtaactatcgtcttgagtccaacccggtaagacacgacttatcgccactggcagcagccactggtaacaggattagcagagcgaggtatgtaggcggtgctacagagttcttgaagtggtggcctaactacggctacactagaagaacagtatttggtatctgcgctctgctgaagccagttaccttcggaaaaagagttggtagctcttgatccggcaaacaaaccaccgctggtagcggtttttttgtttgcaagcagcagattacgcgcagaaaaaaaggatctcaagaagatcctttgatcttttctacggggtctgacgctcagtggaacgaaaactcacgttaagggattttggtcatgagattatcaaaaaggatcttcacctagatccttttaaattaaaaatgaagttttaaatcaatctaaagtatatatgagtaaacttggtctgacagttaccaatgcttaatcagtgaggcacctatctcagcgatctgtctatttcgttcatccatagttgcctgactccccgtcgtgtagataactacgatacgggagggcttaccatctggccccagtgctgcaatgataccgcgagacccacgctcaccggctccagatttatcagcaataaaccagccagccggaagggccgagcgcagaagtggtcctgcaactttatccgcctccatccagtctattaattgttgccgggaagctagagtaagtagttcgccagttaatagtttgcgcaacgttgttgccattgctacaggcatcgtggtgtcacgctcgtcgtttggtatggcttcattcagctccggttcccaacgatcaaggcgagttacatgatcccccatgttgtgcaaaaaagcggttagctccttcggtcctccgatcgttgtcagaagtaagttggccgcagtgttatcactcatggttatggcagcactgcataattctcttactgtcatgccatccgtaagatgcttttctgtgactggtgagtactcaaccaagtcattctgagaatagtgtatgcggcgaccgagttgctcttgcccggcgtcaatacgggataataccgcgccacatagcagaactttaaaagtgctcatcattggaaaacgttcttcggggcgaaaactctcaaggatcttaccgctgttgagatccagttcgatgtaacccactcgtgcacccaactgatcttcagcatcttttactttcaccagcgtttctgggtgagcaaaaacaggaaggcaaaatgccgcaaaaaagggaataagggcgacacggaaatgttgaatactcatactcttcctttttcaatattattgaagcatttatcagggttattgtctcatgagcggatacatatttgaatgtatttagaaaaataaacaaataggggttccgcgcacatttccccgaaaagtgccacctgacgtc

SEQ ID NO: 36 - protein, 332 aa, Artificial Sequence
  mature CYB5R3-HA
MGAQLSTLGHMVLFPVWFLYSLLMKLFQRSTPAITLESPDIKYPLRLIDREIISHDTRRFRFALPSPQHILGLPVGQHIYLSARIDGNLVVRPYTPISSDDDKGFVDLVIKVYFKDTHPKFPAGGKMSQYLESMQIGDTIEFRGPSGLLVYQGKGKFAIRPDKKSNPIIRTVKSVGMIAGGTGITPMLQVIRAIMKDPDDHTVCHLLFANQTEKDILLRPELEELRNKHSARFKLWYTLDRAPEAWDYGQGFVNEEMIRDHLPPPEEEPLVLMCGPPPMIQYACLPNLDHVGHPTERCFVFAYPYDVPDYAGSGATNFSLLKQAGDVEENPG

SEQ ID NO: 37 - protein, 153 aa, Artificial Sequence
  mature IL2-FLAG
APTSSSTKKTQLQLEHLLLDLQMILNGINNYKNPKLTRMLTFKFYMPKKATELKHLQCLEEELKPLEEVLNLAQSKNFHLRPRDLISNINVIVLELKGSETTFMCEYADETATIVEFLNRWITFCQSIISTLTGGRSSAGEQTGDYKDDDDKA

SEQ ID NO: 38 - protein, 172 aa, Artificial Sequence
  mature IL7-FLAG
DCDIEGKDGKQYESVLMVSIDQLLDSMKEIGSNCLNNEFNFFKRHICDANKEGMFLFRAARKLRQFLKMNSTGDFDLHLLKVSEGTTILLNCTGQVKGRKPAALGEAQPTKSLEENKSLKEQKKLNDLCFLKRLLQEIKTCWNKILMGTKEHGGRSSAGEQTGDYKDDDDKA

SEQ ID NO: 39 - protein, 544 aa, Artificial Sequence
  mature IL12(p70)-FLAG
IWELKKDVYVVELDWYPDAPGEMVVLTCDTPEEDGITWTLDQSSEVLGSGKTLTIQVKEFGDAGQYTCHKGGEVLSHSLLLLHKKEDGIWSTDILKDQKEPKNKTFLRCEAKNYSGRFTCWWLTTISTDLTFSVKSSRGSSDPQGVTCGAATLSAERVRGDNKEYEYSVECQEDSACPAAEESLPIEVMVDAVHKLKYENYTSSFFIRDIIKPDPPKNLQLKPLKNSRQVEVSWEYPDTWSTPHSYFSLTFCVQVQGKSKREKKDRVFTDKTSATVICRKNASISVRAQDRYYSSSWSEWASVPCSKGGSEGGSGSEAGGESSGGRERNLPVATPDPGMFPCLHHSQNLLRAVSNMLQKARQTLEFYPCTSEEIDHEDITKDKTSTVEACLPLELTKNESCLNSRETSFITNGSCLASRKTSFMMALCLSSIYEDLKMYQVEFKTMNAKLLMDPKRQIFLDQNMLAVIDELMQALNFNSETVPQKSSLEEPDFYKTKIKLCILLHAFRIRAVTIDRVMSYLNASGGRSSAGEQTGDYKDDDDKA

SEQ ID NO: 40 - protein, 217 aa, Artificial Sequence
  mature IL12A-FLAG
RNLPVATPDPGMFPCLHHSQNLLRAVSNMLQKARQTLEFYPCTSEEIDHEDITKDKTSTVEACLPLELTKNESCLNSRETSFITNGSCLASRKTSFMMALCLSSIYEDLKMYQVEFKTMNAKLLMDPKRQIFLDQNMLAVIDELMQALNFNSETVPQKSSLEEPDFYKTKIKLCILLHAFRIRAVTIDRVMSYLNASGGRSSAGEQTGDYKDDDDKA

SEQ ID NO: 41 - protein, 326 aa, Artificial Sequence
  mature IL12B-FLAG
IWELKKDVYVVELDWYPDAPGEMVVLTCDTPEEDGITWTLDQSSEVLGSGKTLTIQVKEFGDAGQYTCHKGGEVLSHSLLLLHKKEDGIWSTDILKDQKEPKNKTFLRCEAKNYSGRFTCWWLTTISTDLTFSVKSSRGSSDPQGVTCGAATLSAERVRGDNKEYEYSVECQEDSACPAAEESLPIEVMVDAVHKLKYENYTSSFFIRDIIKPDPPKNLQLKPLKNSRQVEVSWEYPDTWSTPHSYFSLTFCVQVQGKSKREKKDRVFTDKTSATVICRKNASISVRAQDRYYSSSWSEWASVPCSGGRSSAGEQTGDYKDDDDKA

SEQ ID NO: 42 - protein, 153 aa, Artificial Sequence
  mature IL15-FLAG
GIHVFILGCFSAGLPKTEANWVNVISDLKKIEDLIQSMHIDATLYTESDVHPSCKVTAMKCFLLELQVISLESGDASIHDTVENLIILANNSLSSNGNVTESGCKECEELEEKNIKEFLQSFVHIVQMFINTSGGRSSAGEQTGDYKDDDDKA

SEQ ID NO: 43 - protein, 153 aa, Artificial Sequence
  mature IL21-FLAG
QGQDRHMIRMRQLIDIVDQLKNYVNDLVPEFLPAPEDVETNCEWSAFSCFQKAQLKSANTGNNERIINVSIKKLKRKPPSTNAGRRQKHRLTCPSCDSYEKKPPKEFLERFKSLLQKMIHQHLSSRTHGSEDSGGRSSAGEQTGDYKDDDDKA

SEQ ID NO: 44 - protein, 193 aa, Artificial Sequence
  mature IL37-FLAG
VHTSPKVKNLNPKKFSIHDQDHKVLVLDSGNLIAVPDKNYIRPEIFFALASSLSSASAEKGSPILLGVSKGEFCLYCDKDKGQSHPSLQLKKEKLMKLAAQKESARRPFIFYRAQVGSWNMLESAAHPGWFICTSCNCNEPVGVTDKFENRKHIEFSFQPVCKAEMSPSEVSDGGRSSAGEQTGDYKDDDDKA

SEQ ID NO: 45 - protein, 147 aa, Artificial Sequence
  mature GMCSF-FLAG
APARSPSPSTQPWEHVNAIQEARRLLNLSRDTAAEMNETVEVISEMFDLQEPTCLQTRLELYKQGLRGSLTKLKGPLTMMASHYKQHCPPTPETSCATQIITFESFKENLKDFLLVIPFDCWEPVQEGGRSSAGEQTGDYKDDDDKA